European Patent Application EP 4 306 647 A1, published January 17, 2024. Title: Method of manufacturing fused protein. Applicant: Sumitomo Dainippon Pharma Co., Ltd. The sequence listing filed with the application follows.

SEQUENCE LISTING (77 sequences)

SEQ ID NO: 1 - DNA, 2583 bp, Artificial Sequence
  codon-optimized gene of NP_001017963 (hHSP90 alpha)
  CDS (13)..(2577)
aagcttgccaccatgcccccttgcagcggcggcgacggctctaccccacccggaccaagcctgagagatcgcgactgtccagcccagtctgctgagtatcccagggatcggctggacccaaggcccggctctccctctgaggcctccagccctccattcctgagatcccgcgctcctgtgaactggtatcaggagaaggcccaggtgtttctgtggcacctgatggtgagcggctctaccacactgctgtgcctgtggaagcagcctttccatgtgagcgcttttccagtgaccgcctccctggctttcaggcagtctcagggagctggacagcacctgtacaaggatctgcagccctttatcctgctgcggctgctgatgcctgaggagacacagacacaggaccagccaatggaggaggaggaggtggagacattcgcctttcaggctgagatcgcccagctgatgtctctgatcatcaacacattctactccaataaggagatctttctgagggagctgatcagcaattcttccgatgccctggacaagatccggtatgagtctctgaccgatccatctaagctggactccggcaaggagctgcacatcaacctgatccccaataagcaggatcggaccctgacaatcgtggacaccggcatcggcatgacaaaggctgacctgatcaacaatctgggcaccatcgccaagagcggcacaaaggctttcatggaggccctgcaggctggagctgatatctccatgatcggccagttcggcgtgggcttttacagcgcttatctggtggccgagaaggtgaccgtgatcacaaagcataacgacgatgagcagtacgcttgggagagctctgccggcggctcttttaccgtgaggaccgatacaggcgagcctatgggccggggcaccaaagtgatcctgcacctgaaggaggaccagacagagtacctggaggagaggcggatcaaggagatcgtgaagaagcattcccagttcatcggctatccaatcacactgtttgtggagaaggagagggataaggaggtgagcgacgatgaggctgaggagaaggaggacaaggaggaggagaaggagaaggaggagaaggagtctgaggacaagcccgagatcgaggatgtgggctccgacgaggaggaggagaagaaggatggcgacaagaagaagaagaagaagatcaaggagaagtatatcgatcaggaggagctgaataagaccaagcccatctggacacggaaccctgacgatatcaccaatgaggagtacggcgagttctataagtccctgacaaacgattgggaggaccacctggccgtgaagcattttagcgtggagggccagctggagttcagagctctgctgtttgtgcctagacgcgccccattcgacctgtttgagaataggaagaagaagaacaatatcaagctgtacgtgaggcgggtgttcatcatggataactgcgaggagctgatccctgagtatctgaattttatcagaggcgtggtggattctgaggacctgccactgaatatcagcagagagatgctgcagcagtctaagatcctgaaagtgatccgcaagaacctggtgaagaagtgtctggagctgttcaccgagctggctgaggacaaggagaactacaagaagttctatgagcagttttccaagaatatcaagctgggcatccacgaggattcccagaacaggaagaagctgagcgagctgctgcggtactatacctccgccagcggcgatgagatggtgagcctgaaggactactgtacacgcatgaaggagaatcagaagcacatctactatatcaccggcgagacaaaggaccaggtggctaactctgccttcgtggagaggctgcggaagcatggcctggaagtgatctacatgatcgagccaatcgatgagtattgcgtgcagcagctgaaggagtttgagggcaagaccctggtgtccgtgacaaaggagggcctggagctgcctgaggatgaggaggagaagaagaagcaggaggagaagaagaccaagttcgagaatctgtgtaagatcatgaaggatatcctggagaagaaggtggagaaggtggtggtgtctaacagactggtgacctccccctgctgtatcgtgacctctacatacggctggacagctaatatggagagaatcatgaaggcccaggctctgcgcgataactccaccatgggctatatggccgctaagaagcacctggagatcaatcctgaccattctatcatcgagacactgcgccagaaggccgaggctgataagaacgacaagtccgtgaaggacctggtcatcctgctgtacgagacagctctgctgtccagcggctttagcctggaggacccccagacacatgccaacagaatctatcgcatgatcaagctgggcctgggcatcgatgaggacgatcctaccgccgacgatacatctgctgctgtgacagaggagatgccccctctggagggcgacgatgacacctccaggatggaggaggtggactgagaattc

SEQ ID NO: 2 - protein, 854 aa, Artificial Sequence
  Synthetic Construct
MPPCSGGDGSTPPGPSLRDRDCPAQSAEYPRDRLDPRPGSPSEASSPPFLRSRAPVNWYQEKAQVFLWHLMVSGSTTLLCLWKQPFHVSAFPVTASLAFRQSQGAGQHLYKDLQPFILLRLLMPEETQTQDQPMEEEEVETFAFQAEIAQLMSLIINTFYSNKEIFLRELISNSSDALDKIRYESLTDPSKLDSGKELHINLIPNKQDRTLTIVDTGIGMTKADLINNLGTIAKSGTKAFMEALQAGADISMIGQFGVGFYSAYLVAEKVTVITKHNDDEQYAWESSAGGSFTVRTDTGEPMGRGTKVILHLKEDQTEYLEERRIKEIVKKHSQFIGYPITLFVEKERDKEVSDDEAEEKEDKEEEKEKEEKESEDKPEIEDVGSDEEEEKKDGDKKKKKKIKEKYIDQEELNKTKPIWTRNPDDITNEEYGEFYKSLTNDWEDHLAVKHFSVEGQLEFRALLFVPRRAPFDLFENRKKKNNIKLYVRRVFIMDNCEELIPEYLNFIRGVVDSEDLPLNISREMLQQSKILKVIRKNLVKKCLELFTELAEDKENYKKFYEQFSKNIKLGIHEDSQNRKKLSELLRYYTSASGDEMVSLKDYCTRMKENQKHIYYITGETKDQVANSAFVERLRKHGLEVIYMIEPIDEYCVQQLKEFEGKTLVSVTKEGLELPEDEEEKKKQEEKKTKFENLCKIMKDILEKKVEKVVVSNRLVTSPCCIVTSTYGWTANMERIMKAQALRDNSTMGYMAAKKHLEINPDHSIIETLRQKAEADKNDKSVKDLVILLYETALLSSGFSLEDPQTHANRIYRMIKLGLGIDEDDPTADDTSAAVTEEMPPLEGDDDTSRMEEVD

SEQ ID NO: 3 - DNA, 2217 bp, Artificial Sequence
  codon-optimized gene of NP_005339 (hHSP90 alpha)
  CDS (13)..(2211)
aagcttgccaccatgcccgaggagacccagacacaggaccagcctatggaggaggaggaggtggagaccttcgcctttcaggctgagatcgcccagctgatgagcctgatcatcaacacattctactctaataaggagatctttctgagagagctgatcagcaattccagcgatgccctggacaagatccgctatgagtctctgaccgatccatctaagctggactccggcaaggagctgcacatcaacctgatccccaataagcaggataggaccctgacaatcgtggacaccggcatcggcatgacaaaggctgacctgatcaacaatctgggcaccatcgccaagtctggcacaaaggctttcatggaggccctgcaggctggagctgatatctccatgatcggccagttcggcgtgggcttttactccgcctatctggtggccgagaaggtgaccgtgatcacaaagcataacgacgatgagcagtacgcttgggagtcttccgccggcggctcctttaccgtgagaaccgatacaggcgagcctatgggccgcggcaccaaagtgatcctgcacctgaaggaggaccagacagagtacctggaggagaggcggatcaaggagatcgtgaagaagcattcccagttcatcggctatccaatcaccctgtttgtggagaaggagagggataaggaggtgagcgacgatgaggctgaggagaaggaggacaaggaggaggagaaggagaaggaggagaaggagtctgaggacaagccagagatcgaggatgtgggctccgacgaggaggaggagaagaaggatggcgacaagaagaagaagaagaagatcaaggagaagtatatcgatcaggaggagctgaataagaccaagcctatctggacacggaacccagacgatatcaccaatgaggagtacggcgagttctataagtccctgacaaacgattgggaggaccacctggccgtgaagcacttctccgtggagggccagctggagttcagggctctgctgtttgtgccaagacgcgcccccttcgacctgtttgagaacaggaagaagaagaacaacatcaagctgtacgtgaggcgggtgttcatcatggataactgcgaggagctgatccctgagtatctgaacttcatcagaggcgtggtggattccgaggacctgccactgaatatctccagggagatgctgcagcagagcaagatcctgaaagtgatccggaagaacctggtgaagaagtgtctggagctgttcaccgagctggctgaggacaaggagaactacaagaagttctatgagcagtttagcaagaatatcaagctgggcatccacgaggattctcagaacagaaagaagctgtccgagctgctgcgctactatacctccgccagcggcgatgagatggtgagcctgaaggactactgcacacgcatgaaggagaatcagaagcacatctactatatcaccggcgagacaaaggaccaggtggctaactctgccttcgtggagagactgcgcaagcatggcctggaagtgatctacatgatcgagccaatcgatgagtattgcgtgcagcagctgaaggagtttgagggcaagaccctggtgagcgtgacaaaggagggactggagctgccagaggacgaggaggagaagaagaagcaggaggagaagaagaccaagttcgagaacctgtgcaagatcatgaaggatatcctggagaagaaggtggagaaggtggtggtgagcaacagactggtgacctctccctgctgtatcgtgacctctacatacggctggacagctaatatggagaggatcatgaaggcccaggctctgcgggataactccaccatgggctatatggccgctaagaagcacctggagatcaatcctgaccattctatcatcgagacactgcgccagaaggccgaggctgataagaacgacaagtccgtgaaggacctggtcatcctgctgtacgagaccgctctgctgagctctggcttttctctggaggacccccagacacatgccaacaggatctatcggatgatcaagctgggcctgggcatcgatgaggacgatcctaccgccgacgatacaagcgccgctgtgaccgaggagatgccacctctggagggcgacgatgacacatctagaatggaggaggtggactgagaattc

SEQ ID NO: 4 - protein, 732 aa, Artificial Sequence
  Synthetic Construct
MPEETQTQDQPMEEEEVETFAFQAEIAQLMSLIINTFYSNKEIFLRELISNSSDALDKIRYESLTDPSKLDSGKELHINLIPNKQDRTLTIVDTGIGMTKADLINNLGTIAKSGTKAFMEALQAGADISMIGQFGVGFYSAYLVAEKVTVITKHNDDEQYAWESSAGGSFTVRTDTGEPMGRGTKVILHLKEDQTEYLEERRIKEIVKKHSQFIGYPITLFVEKERDKEVSDDEAEEKEDKEEEKEKEEKESEDKPEIEDVGSDEEEEKKDGDKKKKKKIKEKYIDQEELNKTKPIWTRNPDDITNEEYGEFYKSLTNDWEDHLAVKHFSVEGQLEFRALLFVPRRAPFDLFENRKKKNNIKLYVRRVFIMDNCEELIPEYLNFIRGVVDSEDLPLNISREMLQQSKILKVIRKNLVKKCLELFTELAEDKENYKKFYEQFSKNIKLGIHEDSQNRKKLSELLRYYTSASGDEMVSLKDYCTRMKENQKHIYYITGETKDQVANSAFVERLRKHGLEVIYMIEPIDEYCVQQLKEFEGKTLVSVTKEGLELPEDEEEKKKQEEKKTKFENLCKIMKDILEKKVEKVVVSNRLVTSPCCIVTSTYGWTANMERIMKAQALRDNSTMGYMAAKKHLEINPDHSIIETLRQKAEADKNDKSVKDLVILLYETALLSSGFSLEDPQTHANRIYRMIKLGLGIDEDDPTADDTSAAVTEEMPPLEGDDDTSRMEEVD

SEQ ID NO: 5 - DNA, 2220 bp, Artificial Sequence
  codon-optimized gene of NP_001233750 (chHSP90 alpha)
  CDS (13)..(2214)
aagcttgccaccatgcccgaggagacccagacacaggaccagcctatggaggaggaggaggtggagaccttcgcctttcaggctgagatcgcccagctgatgagcctgatcatcaacacattctactctaataaggagatctttctgagagagctgatctccaattccagcgatgctctggacaagatccgctatgagagcctgaccgatccatctaagctggactccggcaaggagctgcacatcaacatcatccccaataagcaggataggaccctgacaatcgtggacaccggcatcggcatgacaaaggctgacctgatcaacaatctgggcaccatcgccaagagcggcacaaaggctttcatggaggccctgcaggctggagctgatatctctatgatcggccagttcggcgtgggcttttacaccgcttatctggtggccgagaaggtgaccgtgatcacaaagcataacgacgatgagcagtacgcttgggagtcttccgccggaggctcctttaccgtgaggaccgatacaggcgagcctatgggccggggcaccaaagtgatcctgcacctgaaggaggaccagacagagtacatggaggagaggcggatcaaggagatcgtgaagaagcatagccagttcatcggctatccaatcaccctgtttgtggagaaggagagagataaggaggtgtctgacgatgaggctgaggagaaggaggacaaggaggaggagaaggagaaggaggagaagggcatcgacgataagccagagatcgaggatgtgggcagcgacgaggaggaggaggagaagaaggatggcgacaagaagaagaagaagaagatcaaggagaagtacatcgaccaggaggagctgaataagaccaagcctatctggacacgcaacccagacgatatcaccaatgaggagtacggcgagttctataagtctctgacaaacgattgggaggagcacctggccgtgaagcatttttccgtggagggccagctggagttcagagctctgctgtttgtgccaagacgcgcccccttcgacctgtttgagaacaggaagaagaagaacaacatcaagctgtacgtgaggcgggtgttcatcatggataactgcgaggagctgttccctgagtatctgaacttcatcaggggcgtggtggatagcgaggacctgccactgaatatctcccgggagatcctgcagcagagcaagatcctgaaagtgatcagaaagaacctggtgcgcaagtgtctggagctgtttcacgagctggctgaggacaaggagaactacaagaagttctatgagcagttttctaagaatatcaagctgggcatccatgaggattctcagaacaggaagaagctgtccgagctgctgcggtactatacctccgccagcggcgatgagatggtgtctctgaaggactactgcacaaggatgaaggagaatcagaagcacatctatttcatcaccggcgagacaaaggaccaggtggctaactccgcctttgtggagagactgcgcaagcatggcctggaagtgatctacatgatcgagccaatcgatgagtattgcgtgcagcagctgaaggagttcgagggcaagaccctggtgtctgtgacaaaggagggactggagctgccagaggacgaggaggagaagaagaagcaggaggagaagaagaccaagtttgagaacctgtgcaagatcatgaaggatatcctggagaagaaggtggagaaggtggtggtgagcaacaggctggtgacctctccctgctgtatcgtgacctccacatacggctggacagccaatatggagagaatcatcaaggcccaggctctgcgcgataacagcaccatgggctatatggccgctaagaagcacctggagatcaatcctgaccattccatcatcgagacactgcggcagaaggccgaggctgataagaacgacaagagcgtgaaggacctggtcatcctgctgtacgagaccgctctgctgagctctggcttctccctggaggacccccagacacacgccaacaggatctatcggatgatcaagctgggcctgggcatcgatgaggacgatcctaccgtggacgatacatctgccgctgtgaccgaggagatgccacctctggagggcgacgatgacacatccagaatggaggaggtggactgagaattc

SEQ ID NO: 6 - protein, 733 aa, Artificial Sequence
  Synthetic Construct
MPEETQTQDQPMEEEEVETFAFQAEIAQLMSLIINTFYSNKEIFLRELISNSSDALDKIRYESLTDPSKLDSGKELHINIIPNKQDRTLTIVDTGIGMTKADLINNLGTIAKSGTKAFMEALQAGADISMIGQFGVGFYTAYLVAEKVTVITKHNDDEQYAWESSAGGSFTVRTDTGEPMGRGTKVILHLKEDQTEYMEERRIKEIVKKHSQFIGYPITLFVEKERDKEVSDDEAEEKEDKEEEKEKEEKGIDDKPEIEDVGSDEEEEEKKDGDKKKKKKIKEKYIDQEELNKTKPIWTRNPDDITNEEYGEFYKSLTNDWEEHLAVKHFSVEGQLEFRALLFVPRRAPFDLFENRKKKNNIKLYVRRVFIMDNCEELFPEYLNFIRGVVDSEDLPLNISREILQQSKILKVIRKNLVRKCLELFHELAEDKENYKKFYEQFSKNIKLGIHEDSQNRKKLSELLRYYTSASGDEMVSLKDYCTRMKENQKHIYFITGETKDQVANSAFVERLRKHGLEVIYMIEPIDEYCVQQLKEFEGKTLVSVTKEGLELPEDEEEKKKQEEKKTKFENLCKIMKDILEKKVEKVVVSNRLVTSPCCIVTSTYGWTANMERIIKAQALRDNSTMGYMAAKKHLEINPDHSIIETLRQKAEADKNDKSVKDLVILLYETALLSSGFSLEDPQTHANRIYRMIKLGLGIDEDDPTVDDTSAAVTEEMPPLEGDDDTSRMEEVD

SEQ ID NO: 7 - DNA, 2193 bp, Artificial Sequence
  codon-optimized gene of NP_001258899 (hHSP90 beta)
  CDS (13)..(2187)
aagcttgccaccatgcccgaggaggtgcaccatggcgaggaggaggtggagaccttcgcctttcaggctgagatcgcccagctgatgtccctgatcatcaacacattctacagcaataaggagatctttctgagggagctgatcagcaatgcttctgacgccctggataagatccggtatgagtccctgaccgacccttctaagctggattccggcaaggagctgaagatcgacatcatcccaaacccccaggagaggaccctgacactggtggacaccggcatcggcatgacaaaggctgatctgatcaacaatctgggcaccatcgccaagagcggcacaaaggctttcatggaggccctgcaggctggagctgatatctccatgatcggccagttcggcgtgggcttttactccgcctatctggtggccgagaaggtggtggtcatcaccaagcacaacgacgatgagcagtacgcttgggagtccagcgccggaggcagcttcacagtgagggctgaccacggagagccaatcggaaggggcaccaaagtgatcctgcatctgaaggaggatcagacagagtatctggaggagaggcgggtgaaggaggtggtgaagaagcatagccagtttatcggctaccctatcaccctgtatctggagaaggagcgggagaaggagatctctgacgatgaggccgaggaggagaagggcgagaaggaggaggaggacaaggacgatgaggagaagccaaagatcgaggacgtgggcagcgatgaggaggacgattctggcaaggacaagaagaagaagaccaagaagatcaaggagaagtacatcgatcaggaggagctgaacaagaccaagcctatctggacaaggaatccagacgatatcacccaggaggagtacggcgagttctataagagcctgacaaatgactgggaggatcacctggccgtgaagcatttttctgtggagggccagctggagttccgggctctgctgtttatccccagacgcgcccctttcgacctgtttgagaacaagaagaagaagaacaacatcaagctgtacgtgaggcgggtgttcatcatggactcttgcgatgagctgatccccgagtatctgaacttcatcagaggcgtggtggactccgaggatctgcctctgaacatctccagagagatgctgcagcagagcaagatcctgaaagtgatccgcaagaatatcgtgaagaagtgtctggagctgttttccgagctggctgaggacaaggagaactacaagaagttctatgaggcctttagcaagaatctgaagctgggcatccacgaggactctaccaacagacgcaggctgtccgagctgctgagataccatacctcccagagcggcgatgagatgacatctctgtccgagtacgtgtcccgcatgaaggagacccagaagtccatctactatatcacaggcgagagcaaggagcaggtggctaactctgccttcgtggagcgggtgagaaagcgcggctttgaggtggtgtacatgaccgagccaatcgacgagtattgcgtgcagcagctgaaggagttcgatggcaagtccctggtgagcgtgacaaaggagggactggagctgccagaggacgaggaggagaagaagaagatggaggagtctaaggctaagtttgagaacctgtgcaagctgatgaaggagatcctggataagaaggtggagaaggtgaccatctctaacagactggtgtcttccccatgctgtatcgtgacctccacatacggctggaccgctaatatggagagaatcatgaaggcccaggctctgcgcgacaactccacaatgggctatatgatggccaagaagcacctggagatcaatcctgatcatccaatcgtggagaccctgaggcagaaggctgaggctgacaagaacgataaggctgtgaaggacctggtggtgctgctgttcgagaccgccctgctgagctctggctttagcctggaggatccccagacacactctaataggatctaccggatgatcaagctgggcctgggcatcgacgaggatgaggtggctgctgaggagccaaacgctgctgtgccagacgagatcccacctctggagggcgacgaggatgcttctcgcatggaggaggtggattgagaattc

SEQ ID NO: 8 - protein, 724 aa, Artificial Sequence
  Synthetic Construct
MPEEVHHGEEEVETFAFQAEIAQLMSLIINTFYSNKEIFLRELISNASDALDKIRYESLTDPSKLDSGKELKIDIIPNPQERTLTLVDTGIGMTKADLINNLGTIAKSGTKAFMEALQAGADISMIGQFGVGFYSAYLVAEKVVVITKHNDDEQYAWESSAGGSFTVRADHGEPIGRGTKVILHLKEDQTEYLEERRVKEVVKKHSQFIGYPITLYLEKEREKEISDDEAEEEKGEKEEEDKDDEEKPKIEDVGSDEEDDSGKDKKKKTKKIKEKYIDQEELNKTKPIWTRNPDDITQEEYGEFYKSLTNDWEDHLAVKHFSVEGQLEFRALLFIPRRAPFDLFENKKKKNNIKLYVRRVFIMDSCDELIPEYLNFIRGVVDSEDLPLNISREMLQQSKILKVIRKNIVKKCLELFSELAEDKENYKKFYEAFSKNLKLGIHEDSTNRRRLSELLRYHTSQSGDEMTSLSEYVSRMKETQKSIYYITGESKEQVANSAFVERVRKRGFEVVYMTEPIDEYCVQQLKEFDGKSLVSVTKEGLELPEDEEEKKKMEESKAKFENLCKLMKEILDKKVEKVTISNRLVSSPCCIVTSTYGWTANMERIMKAQALRDNSTMGYMMAKKHLEINPDHPIVETLRQKAEADKNDKAVKDLVVLLFETALLSSGFSLEDPQTHSNRIYRMIKLGLGIDEDEVAAEEPNAAVPDEIPPLEGDEDASRMEEVD

SEQ ID NO: 9 - DNA, 2049 bp, Artificial Sequence
  codon-optimized gene of NP_001258900 (hHSP90 beta)
  CDS (13)..(2043)
aagcttgccaccatgcctgaggaggtgcaccatggcgaggaggaggtggagaccttcgcctttcaggctgagatcgcccagctgatgtccctgatcatcaacacattctacagcaataaggagatctttctgagggagctgatcagcaatgcttctgacgccctggataagatccggtatgagtccctgaccgacccatctaagctggattccggcaaggagctgaagatcgacatctccatgatcggccagttcggcgtgggcttttactccgcctatctggtggccgagaaggtggtggtcatcaccaagcacaacgacgatgagcagtacgcttgggagtccagcgccggaggcagcttcacagtgagggctgaccacggagagccaatcggaaggggcaccaaagtgatcctgcatctgaaggaggatcagacagagtatctggaggagaggcgggtgaaggaggtggtgaagaagcatagccagtttatcggctacccaatcaccctgtatctggagaaggagagggagaaggagatctctgacgatgaggccgaggaggagaagggcgagaaggaggaggaggacaaggacgatgaggagaagcccaagatcgaggacgtgggcagcgatgaggaggacgattctggcaaggacaagaagaagaagaccaagaagatcaaggagaagtacatcgatcaggaggagctgaacaagaccaagccaatctggacaaggaatcccgacgatatcacccaggaggagtacggcgagttctataagagcctgacaaatgactgggaggatcacctggccgtgaagcatttttctgtggagggccagctggagttccgggctctgctgtttatccctagacgcgccccattcgacctgtttgagaacaagaagaagaagaacaacatcaagctgtacgtgaggcgggtgttcatcatggactcttgcgatgagctgatccctgagtatctgaacttcatcagaggcgtggtggactccgaggatctgccactgaacatctccagagagatgctgcagcagagcaagatcctgaaagtgatccgcaagaatatcgtgaagaagtgtctggagctgttctccgagctggctgaggataaggagaactacaagaagttctatgaggcctttagcaagaatctgaagctgggcatccacgaggactctaccaacagacgcaggctgtccgagctgctgagataccatacctcccagagcggcgatgagatgacatctctgtccgagtacgtgtcccgcatgaaggagacccagaagtccatctactatatcacaggcgagagcaaggagcaggtggctaactctgccttcgtggagcgggtgagaaagcgcggctttgaggtggtgtacatgaccgagcccatcgacgagtattgcgtgcagcagctgaaggagttcgatggcaagtccctggtgagcgtgacaaaggagggcctggagctgcctgaggacgaggaggagaagaagaagatggaggagtctaaggctaagtttgagaacctgtgcaagctgatgaaggagatcctggataagaaggtggagaaggtgaccatctctaacagactggtgtcttccccctgctgtatcgtgacctccacatacggctggaccgctaatatggagagaatcatgaaggcccaggctctgcgcgacaactccacaatgggctatatgatggccaagaagcacctggagatcaatccagatcatcccatcgtggagacactgcgccagaaggccgaggctgacaagaacgataaggctgtgaaggacctggtggtgctgctgttcgagaccgccctgctgagctctggctttagcctggaggatcctcagacacactctaataggatctaccggatgatcaagctgggcctgggcatcgacgaggatgaggtggctgctgaggagccaaacgctgctgtgcctgacgagatcccacctctggagggcgacgaggatgcttccaggatggaggaggtggattgagaattc

SEQ ID NO: 10 - protein, 676 aa, Artificial Sequence
  Synthetic Construct
MPEEVHHGEEEVETFAFQAEIAQLMSLIINTFYSNKEIFLRELISNASDALDKIRYESLTDPSKLDSGKELKIDISMIGQFGVGFYSAYLVAEKVVVITKHNDDEQYAWESSAGGSFTVRADHGEPIGRGTKVILHLKEDQTEYLEERRVKEVVKKHSQFIGYPITLYLEKEREKEISDDEAEEEKGEKEEEDKDDEEKPKIEDVGSDEEDDSGKDKKKKTKKIKEKYIDQEELNKTKPIWTRNPDDITQEEYGEFYKSLTNDWEDHLAVKHFSVEGQLEFRALLFIPRRAPFDLFENKKKKNNIKLYVRRVFIMDSCDELIPEYLNFIRGVVDSEDLPLNISREMLQQSKILKVIRKNIVKKCLELFSELAEDKENYKKFYEAFSKNLKLGIHEDSTNRRRLSELLRYHTSQSGDEMTSLSEYVSRMKETQKSIYYITGESKEQVANSAFVERVRKRGFEVVYMTEPIDEYCVQQLKEFDGKSLVSVTKEGLELPEDEEEKKKMEESKAKFENLCKLMKEILDKKVEKVTISNRLVSSPCCIVTSTYGWTANMERIMKAQALRDNSTMGYMMAKKHLEINPDHPIVETLRQKAEADKNDKAVKDLVVLLFETALLSSGFSLEDPQTHSNRIYRMIKLGLGIDEDEVAAEEPNAAVPDEIPPLEGDEDASRMEEVD

SEQ ID NO: 11 - DNA, 2163 bp, Artificial Sequence
  codon-optimized gene of  NP_001258901 (hHSP90 beta)
  CDS (13)..(2157)
aagcttgccaccatgcccgaggaggtgcaccatggcgaggaggaggtggagaccttcgcctttcaggctgagatcgcccagctgatgtccctgatcatcaacacattctacagcaataaggagatctttctgagggagctgatcagcaatgcttctgacgccctggataagatccggtatgagtctctgaccgacccttctaagctggattccggcaaggagctgaagatcgacatcatcccaaacccccaggagaggaccctgacactggtggacaccggcatcggcatgacaaaggctgatctgatcaacaatctgggcaccatcgccaagagcggcacaaaggctttcatggaggccctgcagttcggcgtgggcttttactctgcttatctggtggccgagaaggtggtggtcatcaccaagcacaacgacgatgagcagtacgcttgggagtccagcgccggaggctcctttacagtgagggctgaccacggagagccaatcggaaggggcaccaaagtgatcctgcatctgaaggaggatcagacagagtatctggaggagaggcgggtgaaggaggtggtgaagaagcatagccagttcatcggctaccctatcaccctgtatctggagaaggagcgggagaaggagatctctgacgatgaggccgaggaggagaagggcgagaaggaggaggaggacaaggacgatgaggagaagccaaagatcgaggacgtgggcagcgatgaggaggacgattctggcaaggacaagaagaagaagaccaagaagatcaaggagaagtacatcgatcaggaggagctgaacaagaccaagcctatctggacaaggaatccagacgatatcacccaggaggagtacggcgagttctataagtctctgacaaatgactgggaggatcacctggccgtgaagcatttttccgtggagggacagctggagttccgggctctgctgtttatccccagacgcgcccctttcgacctgtttgagaacaagaagaagaagaacaacatcaagctgtacgtgaggcgggtgttcatcatggactcttgcgatgagctgatccccgagtatctgaacttcatcagaggcgtggtggactccgaggatctgcctctgaacatctccagagagatgctgcagcagagcaagatcctgaaagtgatccgcaagaatatcgtgaagaagtgtctggagctgttttccgagctggctgaggataaggagaactacaagaagttctatgaggcctttagcaagaatctgaagctgggcatccacgaggactctaccaacagacgcaggctgtccgagctgctgagataccatacctcccagagcggcgatgagatgacatctctgtccgagtacgtgtcccgcatgaaggagacccagaagtccatctactatatcacaggcgagagcaaggagcaggtggctaactctgccttcgtggagcgggtgagaaagcgcggctttgaggtggtgtacatgaccgagccaatcgacgagtattgcgtgcagcagctgaaggagttcgatggcaagtccctggtgagcgtgacaaaggagggactggagctgccagaggacgaggaggagaagaagaagatggaggagtccaaggctaagtttgagaacctgtgcaagctgatgaaggagatcctggataagaaggtggagaaggtgaccatctccaacagactggtgtcttccccatgctgtatcgtgaccagcacatacggctggaccgctaatatggagagaatcatgaaggcccaggctctgcgcgacaacagcacaatgggctatatgatggccaagaagcacctggagatcaatcctgatcatccaatcgtggagaccctgaggcagaaggctgaggctgacaagaacgataaggctgtgaaggacctggtggtgctgctgttcgagaccgccctgctgagctctggctttagcctggaggatccccagacacactctaataggatctaccggatgatcaagctgggcctgggcatcgacgaggatgaggtggctgctgaggagccaaacgctgctgtgccagacgagatcccacctctggagggcgacgaggatgcttcccgcatggaggaggtggattgagaattc

SEQ ID NO: 12 - protein, 714 aa, Artificial Sequence
  Synthetic Construct
MPEEVHHGEEEVETFAFQAEIAQLMSLIINTFYSNKEIFLRELISNASDALDKIRYESLTDPSKLDSGKELKIDIIPNPQERTLTLVDTGIGMTKADLINNLGTIAKSGTKAFMEALQFGVGFYSAYLVAEKVVVITKHNDDEQYAWESSAGGSFTVRADHGEPIGRGTKVILHLKEDQTEYLEERRVKEVVKKHSQFIGYPITLYLEKEREKEISDDEAEEEKGEKEEEDKDDEEKPKIEDVGSDEEDDSGKDKKKKTKKIKEKYIDQEELNKTKPIWTRNPDDITQEEYGEFYKSLTNDWEDHLAVKHFSVEGQLEFRALLFIPRRAPFDLFENKKKKNNIKLYVRRVFIMDSCDELIPEYLNFIRGVVDSEDLPLNISREMLQQSKILKVIRKNIVKKCLELFSELAEDKENYKKFYEAFSKNLKLGIHEDSTNRRRLSELLRYHTSQSGDEMTSLSEYVSRMKETQKSIYYITGESKEQVANSAFVERVRKRGFEVVYMTEPIDEYCVQQLKEFDGKSLVSVTKEGLELPEDEEEKKKMEESKAKFENLCKLMKEILDKKVEKVTISNRLVSSPCCIVTSTYGWTANMERIMKAQALRDNSTMGYMMAKKHLEINPDHPIVETLRQKAEADKNDKAVKDLVVLLFETALLSSGFSLEDPQTHSNRIYRMIKLGLGIDEDEVAAEEPNAAVPDEIPPLEGDEDASRMEEVD

SEQ ID NO: 13 - DNA, 2193 bp, Artificial Sequence
  codon-optimized gene of  XP_003501716 (chHSP90 beta)
  CDS (13)..(2187)
aagcttgccaccatgccagaggaggtgcaccatggcgaggaggaggtggagaccttcgcctttcaggctgagatcgcccagctgatgtccctgatcatcaacacattctacagcaataaggagatctttctgcgcgagctgatcagcaatgcttctgacgccctggataagatcagatatgagtctctgaccgacccctctaagctggattccggcaaggagctgaagatcgacatcatcccaaacccccaggagcgcaccctgacactggtggacaccggcatcggcatgacaaaggctgatctgatcaacaatctgggcaccatcgccaagtccggcacaaaggctttcatggaggccctgcaggctggagctgatatctccatgatcggccagttcggcgtgggcttttactccgcctatctggtggccgagaaggtggtggtcatcaccaagcacaatgacgatgagcagtacgcttgggagtccagcgccggaggctccttcacagtgcgcgctgaccacggagagcctatcggaaggggaaccaaagtgatcctgcatctgaaggaggatcagacagagtatctggaggagaggcgggtgaaggaggtggtgaagaagcattcccagtttatcggctaccctatcaccctgtatctggagaaggagagggagaaggagatcagcgacgatgaggccgaggaggagaagggcgagaaggaggaggaggacaaggacgatgaggagaagccaaagatcgaggacgtgggcagcgatgaggaggacgattctggcaaggacaagaagaagaagaccaagaagatcaaggagaagtacatcgatcaggaggagctgaacaagaccaagcctatctggacacgcaatccagacgatatcacccaggaggagtacggcgacttctataagagcctgacaaatgactgggaggatcacctggccgtgaagcatttttctgtggagggccagctggagttcagggctctgctgtttatccccagacgcgcccctttcgatctgtttgagaacaagaagaagaagaacaacatcaagctgtacgtgaggcgggtgttcatcatggacagctgcgatgagctgatcccagagtatctgaacttcatcagaggcgtggtggactctgaggatctgcccctgaacatctcccgggagatgctgcagcagagcaagatcctgaaagtgatcagaaagaatatcgtgaagaagtgtctggagctgttttccgagctggctgaggacaaggagaactacaagaagttctatgaggcctttagcaagaatctgaagctgggcatccacgaggactctaccaacagacgcaggctgtccgagctgctgcggtaccatacctcccagagcggcgatgagatgacatctctgtccgagtacgtgtccagaatgaaggagacccagaagtccatctactatatcacaggcgagagcaaggagcaggtggctaactctgccttcgtggagagggtgccaaagaggggatttgaggccgtgtacatgaccgagcctatcgacgagtattgcgtgcagcagctgaaggagttcgatggcaagtccctggtgagcgtgacaaaggagggactggagctgccagaggacgaggaggagaagaagaagatggaggagagcaaggccaagtttgagaacctgtgcaagctgatgaaggagatcctggataagaaggtggagaaggtgaccatctctaaccggctggtgtcttccccttgctgtatcgtgacctccacatacggctggaccgctaatatggagcggatcatgaaggcccaggctctgagagacaactctacaatgggctatatgatggccaagaagcacctggagatcaatcctgatcatccaatcgtggagacactgagacagaaggccgaggctgacaagaacgataaggctgtgaaggacctggtggtgctgctgttcgagaccgccctgctgagctctggctttagcctggaggatccacagacacactctaaccggatctacagaatgatcaagctgggcctgggcatcgacgaggatgaggtgaccgctgaggagccatctgccgctgtgccagacgagatcccacctctggagggcgacgaggatgcttccaggatggaggaggtggattgagaattc

SEQ ID NO: 14 - protein, 724 aa, Artificial Sequence
  Synthetic Construct
MPEEVHHGEEEVETFAFQAEIAQLMSLIINTFYSNKEIFLRELISNASDALDKIRYESLTDPSKLDSGKELKIDIIPNPQERTLTLVDTGIGMTKADLINNLGTIAKSGTKAFMEALQAGADISMIGQFGVGFYSAYLVAEKVVVITKHNDDEQYAWESSAGGSFTVRADHGEPIGRGTKVILHLKEDQTEYLEERRVKEVVKKHSQFIGYPITLYLEKEREKEISDDEAEEEKGEKEEEDKDDEEKPKIEDVGSDEEDDSGKDKKKKTKKIKEKYIDQEELNKTKPIWTRNPDDITQEEYGDFYKSLTNDWEDHLAVKHFSVEGQLEFRALLFIPRRAPFDLFENKKKKNNIKLYVRRVFIMDSCDELIPEYLNFIRGVVDSEDLPLNISREMLQQSKILKVIRKNIVKKCLELFSELAEDKENYKKFYEAFSKNLKLGIHEDSTNRRRLSELLRYHTSQSGDEMTSLSEYVSRMKETQKSIYYITGESKEQVANSAFVERVPKRGFEAVYMTEPIDEYCVQQLKEFDGKSLVSVTKEGLELPEDEEEKKKMEESKAKFENLCKLMKEILDKKVEKVTISNRLVSSPCCIVTSTYGWTANMERIMKAQALRDNSTMGYMMAKKHLEINPDHPIVETLRQKAEADKNDKAVKDLVVLLFETALLSSGFSLEDPQTHSNRIYRMIKLGLGIDEDEVTAEEPSAAVPDEIPPLEGDEDASRMEEVD

SEQ ID NO: 15 - DNA, 1155 bp, Artificial Sequence
  codon-optimized gene of  NP_008996 (hCDC37)
  CDS (13)..(1149)
aagcttgccaccatggtggactactccgtgtgggatcacatcgaggtgagcgacgatgaggacgagacacatcctaacatcgatacagccagcctgttcagatggagacaccaggctcgcgtggagaggatggagcagtttcagaaggagaaggaggagctggaccggggctgcagagagtgtaagcggaaggtggccgagtgccagagaaagctgaaggagctggaggtggctgagggcggcaaggctgagctggagagactgcaggctgaggctcagcagctgcggaaggaggagagatcctgggagcagaagctggaggagatgaggaagaaggagaagtctatgccctggaacgtggacaccctgtccaaggatggcttctccaagagcatggtgaataccaagcctgagaagacagaggaggatagcgaggaggtgcgcgagcagaagcacaagacattcgtggagaagtatgagaagcagatcaagcattttggcatgctgaggcggtgggacgatagccagaagtacctgtctgacaacgtgcacctggtgtgcgaggagacagctaattacctggtcatctggtgcatcgatctggaggtggaggagaagtgtgccctgatggagcaggtggctcatcagacaatcgtgatgcagttcatcctggagctggccaagtctctgaaggtggacccacgcgcttgttttaggcagttctttaccaagatcaagacagccgaccggcagtacatggagggcttcaacgatgagctggaggcttttaaggagagggtgcggggcagagccaagctgagaatcgagaaggctatgaaggagtacgaggaggaggagcgcaagaagaggctgggacccggcggcctggaccccgtggaggtgtatgagtccctgccagaggagctgcagaagtgctttgacgtgaaggatgtgcagatgctgcaggacgccatcagcaagatggaccctaccgatgctaagtatcatatgcagaggtgtatcgattctggcctgtgggtgccaaattctaaggcctccgaggctaaggagggagaggaggctggacctggcgaccctctgctggaggctgtgcccaagacaggcgacgagaaggatgtgtctgtgtgagaattc

SEQ ID NO: 16 - protein, 378 aa, Artificial Sequence
  Synthetic Construct
MVDYSVWDHIEVSDDEDETHPNIDTASLFRWRHQARVERMEQFQKEKEELDRGCRECKRKVAECQRKLKELEVAEGGKAELERLQAEAQQLRKEERSWEQKLEEMRKKEKSMPWNVDTLSKDGFSKSMVNTKPEKTEEDSEEVREQKHKTFVEKYEKQIKHFGMLRRWDDSQKYLSDNVHLVCEETANYLVIWCIDLEVEEKCALMEQVAHQTIVMQFILELAKSLKVDPRACFRQFFTKIKTADRQYMEGFNDELEAFKERVRGRAKLRIEKAMKEYEEEERKKRLGPGGLDPVEVYESLPEELQKCFDVKDVQMLQDAISKMDPTDAKYHMQRCIDSGLWVPNSKASEAKEGEEAGPGDPLLEAVPKTGDEKDVSV

SEQ ID NO: 17 - DNA, 1158 bp, Artificial Sequence
  codon-optimized gene of XP_003499785 (chCDC37)
  CDS (13)..(1152)
aagcttgccaccatggtggactactccgtgtgggatcacatcgaggtgagcgacgatgaggacgagacccatcctaacatcgatacagccagcctgttcaggtggaggcaccaggctagggtggagaggatggagcagtttcagaaggagaaggacgagctggatcggggctgcagagagtgtaagcggaaggtggccgagtgccagcgcaagctgagggagctggaggtggctgagggaggaggacaggtggagctggagagactgagggctgaggctcagcagctgaggaaggaggagaggtcctgggagcagaagctggaggacatgagaaagaaggagaagtctatgccctggaacgtggacaccctgtccaaggatggcttctccaagagcatcgtgaatatcaagcctgagaaggccgaggaggatagcgaggaggctcgcgagcagaagcataagacattcgtggagaagtatgagaagcagatcaagcactttggcatgctgcatagatgggacgatagccagaagtacctgtctgacaacgtgcacctggtgtgcgaggagaccgccaattacctggtcatctggtgcatcgatctggaggtggaggagaagtgtgccctgatggagcaggtggctcatcagacaatggtcatgcagttcatcctggagctggccaagtctctgaaggtggacccacgggcttgttttagacagttctttaccaagatcaagacagccgatcagcagtacatggagggcttcaagtatgagctggaggcttttaaggagagggtgcggggaagagctaagctgaggatcgagaaggctatgaaggagtacgaggaggaggagcggaagaagagactgggaccaggaggactggacccagtggaggtgtatgagtccctgccagaggagctgcagaagtgcttcgacgtgaaggatgtgcagatgctgcaggacgccatcagcaagatggaccctaccgatgctaagtttcacatgcagaggtgtatcgattctggcctgtgggtgccaaactctaagtccggcgaggccaaggagggagaggaggctggaccaggcgaccctctgctggaggctgtgccaaaggctggcaatgagaaggacgtgtccgcctgagaattc

SEQ ID NO: 18 - protein, 379 aa, Artificial Sequence
  Synthetic Construct
MVDYSVWDHIEVSDDEDETHPNIDTASLFRWRHQARVERMEQFQKEKDELDRGCRECKRKVAECQRKLRELEVAEGGGQVELERLRAEAQQLRKEERSWEQKLEDMRKKEKSMPWNVDTLSKDGFSKSIVNIKPEKAEEDSEEAREQKHKTFVEKYEKQIKHFGMLHRWDDSQKYLSDNVHLVCEETANYLVIWCIDLEVEEKCALMEQVAHQTMVMQFILELAKSLKVDPRACFRQFFTKIKTADQQYMEGFKYELEAFKERVRGRAKLRIEKAMKEYEEEERKKRLGPGGLDPVEVYESLPEELQKCFDVKDVQMLQDAISKMDPTDAKFHMQRCIDSGLWVPNSKSGEAKEGEEAGPGDPLLEAVPKAGNEKDVSA

SEQ ID NO: 19 - DNA, 1740 bp, Artificial Sequence
  codon-optimized gene of NP_955472 (hHSP60)
  CDS (13)..(1734)
aagcttgccaccatgctgagactgcccacagtgttcagacagatgcgccctgtgagcagggtgctggccccacacctgacccgggcctacgctaaggacgtgaagtttggcgccgatgctagagccctgatgctgcagggagtggacctgctggctgatgctgtggctgtgacaatgggccctaagggccgcaccgtgatcatcgagcagtcttggggctccccaaaggtgacaaaggacggcgtgaccgtggccaagtctatcgacctgaaggataagtataagaacatcggcgccaagctggtgcaggacgtggctaacaatacaaatgaggaggccggcgatggcaccacaacagctaccgtgctggctagatctatcgctaaggagggcttcgagaagatctccaagggcgctaaccctgtggagattagacggggcgtgatgctggctgtggatgctgtgatcgccgagctgaagaagcagtctaagcccgtgacaacccctgaggagatcgctcaggtggccaccatcagcgccaacggcgacaaggagatcggcaatatcatctctgatgctatgaagaaggtgggcagaaagggcgtgatcacagtgaaggacggcaagaccctgaacgatgagctggagatcatcgagggcatgaagttcgaccggggctacatcagcccatattttatcaatacatctaagggccagaagtgcgagtttcaggatgcctacgtgctgctgtccgagaagaagatctccagcatccagagcatcgtgccagctctggagatcgccaacgctcacaggaagcccctggtcatcatcgctgaggacgtggatggcgaggccctgtccaccctggtgctgaataggctgaaggtcggcctgcaggtggtggctgtgaaggctcctggatttggcgacaacagaaagaatcagctgaaggatatggccatcgctacaggcggcgccgtgtttggagaggagggcctgaccctgaacctggaggacgtgcagcctcatgatctgggcaaggtcggcgaagtgatcgtgaccaaggacgatgccatgctgctgaagggcaagggcgacaaggctcagatcgagaagagaatccaggagatcatcgagcagctggatgtgacaaccagcgagtacgagaaggagaagctgaatgagagactggctaagctgtctgatggagtggccgtgctgaaggtgggcggcacaagcgatgtggaggtgaacgagaagaaggacagagtgacagatgctctgaatgccacccgcgccgctgtggaggagggaatcgtgctgggcggcggctgtgctctgctgagatgtatccccgccctggactctctgacccctgctaacgaggatcagaagatcggcatcgagatcatcaagcgcacactgaagatcccagccatgaccatcgctaagaatgctggagtggagggctccctgattgtggagaagatcatgcagtcttccagcgaagtgggctatgacgccatggctggcgatttcgtgaatatggtggagaagggcatcatcgaccccacaaaggtggtgaggacagctctgctggatgctgctggagtggcctccctgctgacaaccgctgaggtggtggtgaccgagatcccaaaggaggagaaggaccccggcatgggcgctatgggcggcatgggcggcggcatgggcggcggcatgttttgagaattc

SEQ ID NO: 20 - protein, 573 aa, Artificial Sequence
  Synthetic Construct
MLRLPTVFRQMRPVSRVLAPHLTRAYAKDVKFGADARALMLQGVDLLADAVAVTMGPKGRTVIIEQSWGSPKVTKDGVTVAKSIDLKDKYKNIGAKLVQDVANNTNEEAGDGTTTATVLARSIAKEGFEKISKGANPVEIRRGVMLAVDAVIAELKKQSKPVTTPEEIAQVATISANGDKEIGNIISDAMKKVGRKGVITVKDGKTLNDELEIIEGMKFDRGYISPYFINTSKGQKCEFQDAYVLLSEKKISSIQSIVPALEIANAHRKPLVIIAEDVDGEALSTLVLNRLKVGLQVVAVKAPGFGDNRKNQLKDMAIATGGAVFGEEGLTLNLEDVQPHDLGKVGEVIVTKDDAMLLKGKGDKAQIEKRIQEIIEQLDVTTSEYEKEKLNERLAKLSDGVAVLKVGGTSDVEVNEKKDRVTDALNATRAAVEEGIVLGGGCALLRCIPALDSLTPANEDQKIGIEIIKRTLKIPAMTIAKNAGVEGSLIVEKIMQSSSEVGYDAMAGDFVNMVEKGIIDPTKVVRTALLDAAGVASLLTTAEVVVTEIPKEEKDPGMGAMGGMGGGMGGGMF

SEQ ID NO: 21 - DNA, 1212 bp, Artificial Sequence
  codon-optimized gene of NP_001530 (hHSP40)
  CDS (13)..(1206)
aagcttgccaccatggtgaaggagacaacatactatgacgtgctgggcgtgaagccaaacgccacccaggaggagctgaagaaggcctaccggaagctggctctgaagtatcaccccgataagaaccctaatgagggcgagaagttcaagcagatctctcaggcctacgaggtgctgtccgacgctaagaagagagagctgtatgataagggcggcgagcaggccatcaaggagggcggcgccggcggcggctttggctctcccatggacatctttgatatgttctttgggggcgggggaagaatgcagagagagaggcggggcaagaatgtggtgcatcagctgtccgtgaccctggaggacctgtacaacggcgccacacggaagctggctctgcagaagaatgtgatctgcgataagtgtgagggcagaggcggcaagaagggcgctgtggagtgctgtcctaactgccgcggcaccggcatgcagatcagaatccaccagatcggcccaggcatggtgcagcagatccagagcgtgtgcatggagtgtcagggccatggcgagcggatcagccctaaggacagatgcaagtcttgtaatggccgcaagatcgtgagggagaagaagatcctggaggtgcacatcgacaagggcatgaaggatggccagaagatcacattccatggcgagggcgaccaggagccaggcctggagccaggcgatatcatcatcgtgctggaccagaaggatcacgccgtgttcaccagacgcggcgaggacctgtttatgtgcatggatatccagctggtggaggctctgtgtggctttcagaagccaatctccacactggacaaccgcaccatcgtgatcacaagccaccccggccagatcgtgaagcatggcgatatcaagtgcgtgctgaatgagggcatgcctatctacaggcggccatatgagaagggccgcctgatcatcgagttcaaggtgaactttcccgagaatggcttcctgtcccctgataagctgagcctgctggagaagctgctgccagagaggaaggaggtggaggagacagacgagatggatcaggtggagctggtggactttgatcccaaccaggagagacgcaggcattacaatggcgaggcctatgaggacgatgagcaccatcctaggggcggcgtgcagtgtcagacatcttgagaattc

SEQ ID NO: 22 - protein, 397 aa, Artificial Sequence
  Synthetic Construct
MVKETTYYDVLGVKPNATQEELKKAYRKLALKYHPDKNPNEGEKFKQISQAYEVLSDAKKRELYDKGGEQAIKEGGAGGGFGSPMDIFDMFFGGGGRMQRERRGKNVVHQLSVTLEDLYNGATRKLALQKNVICDKCEGRGGKKGAVECCPNCRGTGMQIRIHQIGPGMVQQIQSVCMECQGHGERISPKDRCKSCNGRKIVREKKILEVHIDKGMKDGQKITFHGEGDQEPGLEPGDIIIVLDQKDHAVFTRRGEDLFMCMDIQLVEALCGFQKPISTLDNRTIVITSHPGQIVKHGDIKCVLNEGMPIYRRPYEKGRLIIEFKVNFPENGFLSPDKLSLLEKLLPERKEVEETDEMDQVELVDFDPNQERRRHYNGEAYEDDEHHPRGGVQCQTS

SEQ ID NO: 23 - DNA, 327 bp, Artificial Sequence
  codon-optimized gene of NP_002148 (hHSP10)
  CDS (13)..(321)
aagcttgccaccatggccggccaggctttcagaaagtttctgccactgtttgacagggtgctggtggagagatctgctgctgagacagtgacaaagggcggcatcatgctgcccgagaagtcccagggcaaggtgctgcaggctacagtggtggctgtgggctccggcagcaagggcaagggcggcgagatccagcccgtgtccgtgaaagtgggcgataaggtgctgctgcctgagtacggcggcacaaaggtggtgctggacgataaggactatttcctgtttcgcgacggcgatatcctgggcaagtacgtggattgagaattc

SEQ ID NO: 24 - protein, 102 aa, Artificial Sequence
  Synthetic Construct
MAGQAFRKFLPLFDRVLVERSAAETVTKGGIMLPEKSQGKVLQATVVAVGSGSKGKGGEIQPVSVKVGDKVLLPEYGGTKVVLDDKDYFLFRDGDILGKYVD

SEQ ID NO: 25 - DNA, 2595 bp, Artificial Sequence
  codon-optimized gene of NP_006635 (hHSP110)
  CDS (13)..(2589)
aagcttgccaccatgtccgtggtgggcctggatgtgggcagccagtcttgttacattgctgtggctagagccggcggcattgagacaatcgccaacgagttcagcgacaggtgcaccccatctgtgatctcctttggcagcaagaatcggaccatcggcgtggccgctaagaaccagcagatcacccacgctaacaatacagtgtctaatttcaagaggtttcatggccgggccttcaacgatccctttatccagaaggagaaggagaatctgtcctacgacctggtgcctctgaagaacggcggcgtgggcatcaaagtgatgtatatgggcgaggagcatctgttctccgtcgagcagatcaccgctatgctgctgacaaagctgaaggagacagccgagaatagcctgaagaagcccgtgacagactgtgtgatctctgtgccttccttctttaccgacgctgagaggcggtctgtgctggatgccgctcagatcgtgggcctgaattgcctgagactgatgaacgatatgacagctgtggccctgaactacggcatctataagcaggacctgccttccctggatgagaagccacgcatcgtggtgttcgtggacatgggccactccgctttccaggtgagcgcttgtgcctttaataagggcaagctgaaggtgctgggcacagccttcgatccatttctgggcggcaagaactttgacgagaagctggtggagcatttctgcgccgagtttaagaccaagtacaagctggatgctaagagcaagatcagagccctgctgcgcctgtatcaggagtgcgagaagctgaagaagctgatgtccagcaattctaccgacctgcccctgaatatcgagtgtttcatgaacgacaaggatgtgagcggcaagatgaaccgctctcagtttgaggagctgtgcgctgagctgctgcagaagatcgaggtgcctctgtatagcctgctggagcagacacacctgaaggtggaggatgtgtctgccgtggagatcgtgggcggcgctaccagaatcccagccgtgaaggagcgcatcgctaagttctttggcaaggacatctccaccacactgaacgctgatgaggctgtggccaggggctgtgctctgcagtgtgctatcctgtctcccgctttcaaggtgcgggagttttccgtgacagacgccgtgccattccccatctccctgatctggaatcatgacagcgaggataccgagggcgtgcacgaggtgttctccaggaaccatgccgctcctttctccaaggtgctgacctttctgagacgcggcccattcgagctggaggccttttacagcgatccccagggcgtgccttatccagaggctaagatcggccgcttcgtggtgcagaatgtgagcgcccagaaggacggcgagaagtctagggtgaaggtgaaggtgcgggtgaacacacacggcatctttaccatcagcacagcttctatggtggagaaggtgcccaccgaggagaacgagatgtcttccgaggccgacatggagtgtctgaatcagaggccccctgagaacccagacacagataagaatgtgcagcaggataactctgaggctggcacccagccacaggtgcagacagatgctcagcagacctcccagagcccaccctctcctgagctgacatccgaggagaataagatcccagacgctgataaggccaacgagaagaaggtggatcagcctccagaggctaagaagcccaagatcaaggtggtgaatgtggagctgcctatcgaggccaacctggtgtggcagctgggcaaggacctgctgaatatgtacatcgagacagagggcaagatgatcatgcaggacaagctggagaaggagagaaatgatgctaagaacgccgtggaggagtacgtgtatgagttccgcgataagctgtgcggcccttatgagaagttcatctgtgagcaggaccatcagaactttctgcggctgctgaccgagacagaggactggctgtacgaggagggcgaggatcaggctaagcaggcctatgtggacaagctggaggagctgatgaagatcggcaccccagtgaaggtgaggttccaggaggctgaggagcggcccaagatgtttgaggagctgggccagagactgcagcactacgccaagatcgccgctgactttcgcaataaggatgagaagtataaccatatcgatgagtccgagatgaagaaggtggagaagagcgtgaatgaagtgatggagtggatgaacaatgtgatgaacgctcaggccaagaagagcctggaccaggaccccgtggtgagggctcaggagatcaagacaaagatcaaggagctgaacaatacatgtgagcctgtggtgacccagcccaagcctaagatcgagtctccaaagctggagcggaccccaaacggccccaatatcgacaagaaggaggaggacctggaggataagaacaattttggagctgagccccctcaccagaatggagagtgctacccaaacgagaagaactccgtgaacatggacctggattgagaattc

SEQ ID NO: 26 - protein, 858 aa, Artificial Sequence
  Synthetic Construct
MSVVGLDVGSQSCYIAVARAGGIETIANEFSDRCTPSVISFGSKNRTIGVAAKNQQITHANNTVSNFKRFHGRAFNDPFIQKEKENLSYDLVPLKNGGVGIKVMYMGEEHLFSVEQITAMLLTKLKETAENSLKKPVTDCVISVPSFFTDAERRSVLDAAQIVGLNCLRLMNDMTAVALNYGIYKQDLPSLDEKPRIVVFVDMGHSAFQVSACAFNKGKLKVLGTAFDPFLGGKNFDEKLVEHFCAEFKTKYKLDAKSKIRALLRLYQECEKLKKLMSSNSTDLPLNIECFMNDKDVSGKMNRSQFEELCAELLQKIEVPLYSLLEQTHLKVEDVSAVEIVGGATRIPAVKERIAKFFGKDISTTLNADEAVARGCALQCAILSPAFKVREFSVTDAVPFPISLIWNHDSEDTEGVHEVFSRNHAAPFSKVLTFLRRGPFELEAFYSDPQGVPYPEAKIGRFVVQNVSAQKDGEKSRVKVKVRVNTHGIFTISTASMVEKVPTEENEMSSEADMECLNQRPPENPDTDKNVQQDNSEAGTQPQVQTDAQQTSQSPPSPELTSEENKIPDADKANEKKVDQPPEAKKPKIKVVNVELPIEANLVWQLGKDLLNMYIETEGKMIMQDKLEKERNDAKNAVEEYVYEFRDKLCGPYEKFICEQDHQNFLRLLTETEDWLYEEGEDQAKQAYVDKLEELMKIGTPVKVRFQEAEERPKMFEELGQRLQHYAKIAADFRNKDEKYNHIDESEMKKVEKSVNEVMEWMNNVMNAQAKKSLDQDPVVRAQEIKTKIKELNNTCEPVVTQPKPKIESPKLERTPNGPNIDKKEEDLEDKNNFGAEPPHQNGECYPNEKNSVNMDLD

SEQ ID NO: 27 - DNA, 1767 bp, Artificial Sequence
  codon-optimized gene of chHSP70
  CDS (13)..(1761)
aagcttgccaccatggctaagaacaccgccatcggcatcgacctgggcaccacatactcctgcgtgggcgtgttccagcacggcaaggtggagatcatcgccaacgatcagggcaatcggaccacacctagctatgtggcttttaccgacacagagagactgatcggcgatgccgctaagaatcaggtggccctgaacccacagaataccgtgttcgacgctaagagactgatcggccgcaagtttggcgacgccgtggtgcagagcgatatgaagcactggccattccaggtggtgaacgacggcgataagcccaaggtgcaagtgaattacaagggcgagtccaggtccttcttccccgaggagatctccagcatggtgctgacaaagatgaaggagatcgctgaggcctacctgggccatcccgtgaccaacgccgtgatcacagtgcctgcttacttcaacgactctcagcggcaggctaccaaggatgccggcgtgatcgctggcctgaacgtgctgagaatcatcaatgagcctacagccgctgccatcgcctacggcctggacagaaaccgccagggcaagaaggatatctctcagaataagctggctgtgaggcggctgaggaccgcttgcgagagggctaagcggaccctgtcttccagcacacaggccagcctggagatcgactctctgttcgagggcatcgacttctacacctccatcacaagggctcggttcgaggagctgtgctccgacctgtttaggagcaccctggagccagtggagaaggccctgagggacgctaagatggataaggcccagatccatgatctggtgctggtgggaggcagcacacgcatcccaaaggtgcagaagctgctgcaggacttctttaacggcagggatctgaacaagtctatcaatccagacgaggctgtggcttatggagctgctgtgcaggctgctatcctgatgggcgataagtccgagaatgtgcaggacctgctgctgctggatgtggctcctctgagcctgggcctggagaccgctggaggcgtgatgacagctctgatcaagcgcaacagcaccatccccacaaagcagacccagacattcaccacatactctgacaatcagcctggcgtgctgatccaggtgtatgagggcgagagagccatgaccggcgataacaatctgctgggccgcttcgagctgtccggcatcccccctgctccaaggggcgtgccccagatcgaggtgacctttgacatcgatgccaacggcctgaatgtgaccgctacagacaagtctacaggcaaggccaacaagatcaccatcacaaatgataagggcaggctgtccaaggaggagatcgagagaatggtgcaggaggccgagaggtacaaggctgaggacgaggtgcagagagatcgcgtggctgccaagaacgccctggagtcttatgcttttaatatgaagtccgccgtggagggagagggcctgaagggcaagctgtccgaggctgacaagaagaaggtgctggacaagtgccaggaagtgatctcctggctggacagcaacaccctggccgataaggaggagttcgtgcacaagagggaggagctggagagggtgtgctctcctatcatctccggcctgtaccagggagctggagctccaggagctggaggctttggagctcaggctcctaagggagctagcggctctggaccaacaatcgaggaggtggactgagaattc

SEQ ID NO: 28 - protein, 582 aa, Artificial Sequence
  Synthetic Construct
MAKNTAIGIDLGTTYSCVGVFQHGKVEIIANDQGNRTTPSYVAFTDTERLIGDAAKNQVALNPQNTVFDAKRLIGRKFGDAVVQSDMKHWPFQVVNDGDKPKVQVNYKGESRSFFPEEISSMVLTKMKEIAEAYLGHPVTNAVITVPAYFNDSQRQATKDAGVIAGLNVLRIINEPTAAAIAYGLDRNRQGKKDISQNKLAVRRLRTACERAKRTLSSSTQASLEIDSLFEGIDFYTSITRARFEELCSDLFRSTLEPVEKALRDAKMDKAQIHDLVLVGGSTRIPKVQKLLQDFFNGRDLNKSINPDEAVAYGAAVQAAILMGDKSENVQDLLLLDVAPLSLGLETAGGVMTALIKRNSTIPTKQTQTFTTYSDNQPGVLIQVYEGERAMTGDNNLLGRFELSGIPPAPRGVPQIEVTFDIDANGLNVTATDKSTGKANKITITNDKGRLSKEEIERMVQEAERYKAEDEVQRDRVAAKNALESYAFNMKSAVEGEGLKGKLSEADKKKVLDKCQEVISWLDSNTLADKEEFVHKREELERVCSPIISGLYQGAGAPGAGGFGAQAPKGASGSGPTIEEVD

SEQ ID NO: 29 - DNA, 630 bp, Artificial Sequence
  codon-optimized gene of chHSP27
  CDS (13)..(624)
aagcttgccaccatgaccgagaggcgggtgcctttctccctgctgaggtctccatcctgggagccctttcgggactggtacccagctcacagcagactgttcgatcaggcctttggcgtgccaaggctgcctgacgagtggagccagtggttctctgccgctggatggccaggatatgtgaggccactgccagctgctaccgctgagggacctgctgctgtgacactggctgctccagccttttccagggctctgaacaggcagctgtccagcggcgtgagcgagatcaggcagaccgctgacagatggcgcgtgtctctggatgtgaatcatttcgcccctgaggagctgaccgtgaagacaaaggagggcgtggtggagatcacaggcaagcacgaggagagacaggatgagcatggctacatctccagatgctttacccgcaagtatacactgccacctggagtggaccccaccctggtgtcttccagcctgtctcctgagggcaccctgacagtggaggctcctctgccaaaggctgtgacacagtccgccgagatcaccatcccagtgacattcgaggcccgcgctcagatcggcggccccgaggccggcaaggtgtgagaattc

SEQ ID NO: 30 - protein, 203 aa, Artificial Sequence
  Synthetic Construct
MTERRVPFSLLRSPSWEPFRDWYPAHSRLFDQAFGVPRLPDEWSQWFSAAGWPGYVRPLPAATAEGPAAVTLAAPAFSRALNRQLSSGVSEIRQTADRWRVSLDVNHFAPEELTVKTKEGVVEITGKHEERQDEHGYISRCFTRKYTLPPGVDPTLVSSSLSPEGTLTVEAPLPKAVTQSAEITIPVTFEARAQIGGPEAGKV

SEQ ID NO: 31 - DNA, 687 bp, Artificial Sequence
  codon-optimized gene of BDNF precursor
  CDS (1)..(687)
gccccaatgaaggaggctaacatcaggggacagggaggactggcttaccctggcgtgcggacccacggcacactggagtccgtgaatggcccaaaggctggctcccggggcctgaccagcctggctgacacattcgagcatgtgatcgaggagctgctggacgaggatcagaaggtgagacctaacgaggagaacaataaggacgctgatctgtataccagccgcgtgatgctgtccagccaggtgccactggagccacctctgctgtttctgctggaggagtacaagaactatctggatgccgctaatatgtccatgagggtgaggcggcacagcgacccagctagaaggggagagctgtccgtgtgcgattccatcagcgagtgggtgaccgccgctgacaagaagacagctgtggatatgagcggcggcaccgtgacagtgctggagaaggtgcccgtgtctaagggccagctgaagcagtatttctacgagaccaagtgcaaccctatgggctacacaaaggagggctgtaggggcatcgacaagcggcattggaactcccagtgtagaaccacacagtcctatgtgcgcgccctgaccatggactccaagaagaggatcggctggaggttcatccgcatcgatacaagctgcgtgtgcaccctgacaatcaagaggggccgg

SEQ ID NO: 32 - protein, 229 aa, Artificial Sequence
  Synthetic Construct
APMKEANIRGQGGLAYPGVRTHGTLESVNGPKAGSRGLTSLADTFEHVIEELLDEDQKVRPNEENNKDADLYTSRVMLSSQVPLEPPLLFLLEEYKNYLDAANMSMRVRRHSDPARRGELSVCDSISEWVTAADKKTAVDMSGGTVTVLEKVPVSKGQLKQYFYETKCNPMGYTKEGCRGIDKRHWNSQCRTTQSYVRALTMDSKKRIGWRFIRIDTSCVCTLTIKRGR

SEQ ID NO: 33 - DNA, 852 bp, Artificial Sequence
  DNAJB2 HSJ1, HSPF3 AAA09034
  CDS (13)..(846)
aagcttgccaccatggcctcttactatgagatcctggacgtgcccagaagcgcctctgctgacgatatcaagaaggcctacaggcggaaggctctgcagtggcaccccgacaagaaccctgataataaggagtttgctgagaagaagttcaaggaggtggccgaggcttatgaggtgctgtccgacaagcataagagggagatctacgatagatatggccgggagggcctgacaggcacaggcaccggacctagccgggccgaggctggctctggcggccctggcttcaccttcaccttcaggtcccccgaagaggtgtttcgggagttctttggctccggcgacccatttgccgagctgttcgacgatctgggccccttcagcgagctgcagaacagaggctcccgccactctggacccttctttacattttccagctctttccctggccattctgatttttccagctcttccttttccttcagcccaggcgccggcgcttttagatctgtgtccaccagcaccacattcgtgcagggcagacgcatcaccacaaggcggatcatggagaatggacaggagagagtggaggtggaggaggacggccagctgaagtccgtgacaatcaatggcgtgcctgacgatctggccagaggcctggagctgtccagacgcgagcagcagccttctgtgacctctcgctccggcggcacacaggtgcagcagaccccagctagctgccccctggactctgatctgtccgaggacgaggatctgcagctggccatggcttacagcctgtctgagatggaggccgctggcaagaagcccgctgatgtgttctgagaattc

SEQ ID NO: 34 - protein, 277 aa, Artificial Sequence [sequence omitted]

SEQ ID NO: 35 - DNA, 57 bp, Artificial Sequence
  IgG signal sequence 6SVL_B
  CDS (1)..(57)
atgggctggtctctgatcctgctgttcctggtggctgtggctaccagggtgggatcc

SEQ ID NO: 36 - protein, 19 aa, Artificial Sequence
  Synthetic Construct
MGWSLILLFLVAVATRVGS

SEQ ID NO: 37 - DNA, 678 bp, Artificial Sequence
  hFab heavy chain
  CDS (1)..(678)
gaggtgcagctggtgcagagcggagctgaggtgaagaagccaggcgagagcctgaagatctcttgcaagggctccggctacagcttcatgaactattggctgggctgggtgagacagatgcctggcaagggcctggagtggatgggcgacatctaccccggcggcgattaccctacctatagcgagaagtttaaggtgcaggtgaccatctctgccgacaagtctatctccacagcttatctgcagctgtcttccctgaaggcctccgacaccgctatgtactattgcgcccgcagcggcaattacgatgaggtggcttattggggccagggcaccctggtgacagtgagctctgccagcacaaagggcccctccgtgttccctctggctccatccagcaagagcacctctggaggaacagccgctctgggatgtctggtgaaggattacttcccagagcccgtgaccgtgtcttggaactccggcgccctgaccagcggagtgcacacatttccagctgtgctgcagtcttccggcctgtactctctgagctctgtggtgaccgtgccctccagctctctgggcacccagacatatatctgcaacgtgaatcacaagccatctaatacaaaggtggacaagaaggtggagcccaagtcctgtgataagacccataca

SEQ ID NO: 38 - protein, 226 aa, Artificial Sequence
  Synthetic Construct
EVQLVQSGAEVKKPGESLKISCKGSGYSFMNYWLGWVRQMPGKGLEWMGDIYPGGDYPTYSEKFKVQVTISADKSISTAYLQLSSLKASDTAMYYCARSGNYDEVAYWGQGTLVTVSSASTKGPSVFPLAPSSKSTSGGTAALGCLVKDYFPEPVTVSWNSGALTSGVHTFPAVLQSSGLYSLSSVVTVPSSSLGTQTYICNVNHKPSNTKVDKKVEPKSCDKTHT

SEQ ID NO: 39 - DNA, 1518 bp, Artificial Sequence
  BDNF-hFab(H)
  CDS (13)..(1512)
gaattcgccaccatgggctggtctctgatcctgctgttcctggtggctgtggctaccagggtgggatccgccccaatgaaggaggctaacatcaggggacagggaggactggcttaccctggcgtgcggacccacggcacactggagtccgtgaatggcccaaaggctggctcccggggcctgaccagcctggctgacacattcgagcatgtgatcgaggagctgctggacgaggatcagaaggtgagacctaacgaggagaacaataaggacgctgatctgtataccagccgcgtgatgctgtccagccaggtgccactggagccacctctgctgtttctgctggaggagtacaagaactatctggatgccgctaatatgtccatgagggtgaggcggcacagcgacccagctagaaggggagagctgtccgtgtgcgattccatcagcgagtgggtgaccgccgctgacaagaagacagctgtggatatgagcggcggcaccgtgacagtgctggagaaggtgcccgtgtctaagggccagctgaagcagtatttctacgagaccaagtgcaaccctatgggctacacaaaggagggctgtaggggcatcgacaagcggcattggaactcccagtgtagaaccacacagtcctatgtgcgcgccctgaccatggactccaagaagaggatcggctggaggttcatccgcatcgatacaagctgcgtgtgcaccctgacaatcaagaggggccggggaggaggaggatctggaggaggcggctcaggcggcggcggcagcggcggcggcggctctggcggcggcggctccgaggtgcagctggtgcagagcggagctgaggtgaagaagccaggcgagagcctgaagatctcttgcaagggctccggctacagcttcatgaactattggctgggctgggtgagacagatgcctggcaagggcctggagtggatgggcgacatctaccccggcggcgattaccctacctatagcgagaagtttaaggtgcaggtgaccatctctgccgacaagtctatctccacagcttatctgcagctgtcttccctgaaggcctccgacaccgctatgtactattgcgcccgcagcggcaattacgatgaggtggcttattggggccagggcaccctggtgacagtgagctctgccagcacaaagggcccctccgtgttccctctggctccatccagcaagagcacctctggaggaacagccgctctgggatgtctggtgaaggattacttcccagagcccgtgaccgtgtcttggaactccggcgccctgaccagcggagtgcacacatttccagctgtgctgcagtcttccggcctgtactctctgagctctgtggtgaccgtgccctccagctctctgggcacccagacatatatctgcaacgtgaatcacaagccatctaatacaaaggtggacaagaaggtggagcccaagtcctgtgataagacccatacataatctaga

SEQ ID NO: 40 - protein, 499 aa, Artificial Sequence
  Synthetic Construct
MGWSLILLFLVAVATRVGSAPMKEANIRGQGGLAYPGVRTHGTLESVNGPKAGSRGLTSLADTFEHVIEELLDEDQKVRPNEENNKDADLYTSRVMLSSQVPLEPPLLFLLEEYKNYLDAANMSMRVRRHSDPARRGELSVCDSISEWVTAADKKTAVDMSGGTVTVLEKVPVSKGQLKQYFYETKCNPMGYTKEGCRGIDKRHWNSQCRTTQSYVRALTMDSKKRIGWRFIRIDTSCVCTLTIKRGRGGGGSGGGGSGGGGSGGGGSGGGGSEVQLVQSGAEVKKPGESLKISCKGSGYSFMNYWLGWVRQMPGKGLEWMGDIYPGGDYPTYSEKFKVQVTISADKSISTAYLQLSSLKASDTAMYYCARSGNYDEVAYWGQGTLVTVSSASTKGPSVFPLAPSSKSTSGGTAALGCLVKDYFPEPVTVSWNSGALTSGVHTFPAVLQSSGLYSLSSVVTVPSSSLGTQTYICNVNHKPSNTKVDKKVEPKSCDKTHT

SEQ ID NO: 41 - DNA, 657 bp, Artificial Sequence
  hFab light chain
  CDS (1)..(657)
gacatcgtgatgacccagacaccactgtccctgagcgtgaccccaggacagccagcttctatctcctgccgctccagccagtccctggtgcacagcaacggcaatacctacctgcattggtatctgcagaagcctggccagtccccacagctgctgatctacaaggtgtctaacaggttctccggagtgccagaccggtttagcggatctggatccggcaccgatttcacactgaagatctccagggtggaggccgaggatgtgggcgtgtactattgcagccagtctacccacgtgccctggacatttggccagggcaccaaggtggagatcaagcggacagtggccgctccttccgtgttcatctttccccctagcgacgagcagctgaagagcggcaccgcttctgtggtgtgcctgctgaacaatttctaccctagagaggccaaggtgcagtggaaggtggataacgctctgcagtccggcaatagccaggagtctgtgacagagcaggactccaaggatagcacctattctctgtcttccaccctgacactgagcaaggccgactacgagaagcacaaggtgtatgcttgcgaggtgacacatcagggcctgagctctccagtgaccaagtcttttaatcgcggcgagtgt

SEQ ID NO: 42 - protein, 219 aa, Artificial Sequence
  Synthetic Construct
DIVMTQTPLSLSVTPGQPASISCRSSQSLVHSNGNTYLHWYLQKPGQSPQLLIYKVSNRFSGVPDRFSGSGSGTDFTLKISRVEAEDVGVYYCSQSTHVPWTFGQGTKVEIKRTVAAPSVFIFPPSDEQLKSGTASVVCLLNNFYPREAKVQWKVDNALQSGNSQESVTEQDSKDSTYSLSSTLTLSKADYEKHKVYACEVTHQGLSSPVTKSFNRGEC

SEQ ID NO: 43 - DNA, 735 bp, Artificial Sequence
  hFab(L)
  CDS (13)..(729)
gaattcgccaccatgggctggtctctgatcctgctgttcctggtggccgtggctacaagagtgggctccgacatcgtgatgacccagacaccactgtccctgagcgtgaccccaggacagccagcttctatctcctgccgctccagccagtccctggtgcacagcaacggcaatacctacctgcattggtatctgcagaagcctggccagtccccacagctgctgatctacaaggtgtctaacaggttctccggagtgccagaccggtttagcggatctggatccggcaccgatttcacactgaagatctccagggtggaggccgaggatgtgggcgtgtactattgcagccagtctacccacgtgccctggacatttggccagggcaccaaggtggagatcaagcggacagtggccgctccttccgtgttcatctttccccctagcgacgagcagctgaagagcggcaccgcttctgtggtgtgcctgctgaacaatttctaccctagagaggccaaggtgcagtggaaggtggataacgctctgcagtccggcaatagccaggagtctgtgacagagcaggactccaaggatagcacctattctctgtcttccaccctgacactgagcaaggccgactacgagaagcacaaggtgtatgcttgcgaggtgacacatcagggcctgagctctccagtgaccaagtcttttaatcgcggcgagtgttaatctaga

SEQ ID NO: 44 - protein, 238 aa, Artificial Sequence
  Synthetic Construct
MGWSLILLFLVAVATRVGSDIVMTQTPLSLSVTPGQPASISCRSSQSLVHSNGNTYLHWYLQKPGQSPQLLIYKVSNRFSGVPDRFSGSGSGTDFTLKISRVEAEDVGVYYCSQSTHVPWTFGQGTKVEIKRTVAAPSVFIFPPSDEQLKSGTASVVCLLNNFYPREAKVQWKVDNALQSGNSQESVTEQDSKDSTYSLSSTLTLSKADYEKHKVYACEVTHQGLSSPVTKSFNRGEC

SEQ ID NO: 45 - DNA, 3887 bp, Homo sapiens
  CDS (346)..(2910): NM_001017963 WT, CDS 346-2910
gactgcgcaggcgtgctcacctggcgtgctccacccgactgggcgtccgcaggctcctcccccgggtgtggcctccgggcggcatggctgcttcccaggtgatgccggcttcagctagtggggtctagttgaccgttccgcagccgccagggccagcggaaagccggtcagggggaaccgcggcggggctggtgtcatgagcctgaggtgaacttgagggtgcctcctcagcggtctcccgccctgccctgaggggcgccgggaccccaaagagcggaggaagagcgccaccccgacggccaccgcttcggagccagcacgcggggtaccctacggggagcgcggatgcccccgtgttcgggcggggacggctccacccctcctgggccctcccttcgggacagggactgtcccgcccagagtgctgaatacccgcgcgaccgtctggatccccgcccaggaagcccctctgaagcctcctcgccgccgtttctgagaagcagggcacctgttaactggtaccaagaaaaggcccaagtgtttctctggcatctgatggtgtctggatccaccactctactctgtctctggaaacagcccttccacgtctctgcattccctgtcaccgcgtcactggccttcagacagagccaaggtgcagggcaacacctctacaaggatctgcagccatttatattgcttaggctactgatgcctgaggaaacccagacccaagaccaaccgatggaggaggaggaggttgagacgttcgcctttcaggcagaaattgcccagttgatgtcattgatcatcaatactttctactcgaacaaagagatctttctgagagagctcatttcaaattcatcagatgcattggacaaaatccggtatgaaagcttgacagatcccagtaaattagactctgggaaagagctgcatattaaccttataccgaacaaacaagatcgaactctcactattgtggatactggaattggaatgaccaaggctgacttgatcaataaccttggtactatcgccaagtctgggaccaaagcgttcatggaagctttgcaggctggtgcagatatctctatgattggccagttcggtgttggtttttattctgcttatttggttgctgagaaagtaactgtgatcaccaaacataacgatgatgagcagtacgcttgggagtcctcagcagggggatcattcacagtgaggacagacacaggtgaacctatgggtcgtggaacaaaagttatcctacacctgaaagaagaccaaactgagtacttggaggaacgaagaataaaggagattgtgaagaaacattctcagtttattggatatcccattactctttttgtggagaaggaacgtgataaagaagtaagcgatgatgaggctgaagaaaaggaagacaaagaagaagaaaaagaaaaagaagagaaagagtcggaagacaaacctgaaattgaagatgttggttctgatgaggaagaagaaaagaaggatggtgacaagaagaagaagaagaagattaaggaaaagtacatcgatcaagaagagctcaacaaaacaaagcccatctggaccagaaatcccgacgatattactaatgaggagtacggagaattctataagagcttgaccaatgactgggaagatcacttggcagtgaagcatttttcagttgaaggacagttggaattcagagcccttctatttgtcccacgacgtgctccttttgatctgtttgaaaacagaaagaaaaagaacaacatcaaattgtatgtacgcagagttttcatcatggataactgtgaggagctaatccctgaatatctgaacttcattagaggggtggtagactcggaggatctccctctaaacatatcccgtgagatgttgcaacaaagcaaaattttgaaagttatcaggaagaatttggtcaaaaaatgcttagaactctttactgaactggcggaagataaagagaactacaagaaattctatgagcagttctctaaaaacataaagcttggaatacacgaagactctcaaaatcggaagaagctttcagagctgttaaggtactacacatctgcctctggtgatgagatggtttctctcaaggactactgcaccagaatgaaggagaaccagaaacatatctattatatcacaggtgagaccaaggaccaggtagctaactcagcctttgtggaacgtcttcggaaacatggcttagaagtgatctatatgattgagcccattgatgagtactgtgtccaacagctgaaggaatttgaggggaagactttagtgtcagtcaccaaagaaggcctggaacttccagaggatgaagaagagaaaaagaagcaggaagagaaaaaaacaaagtttgagaacctctgcaaaatcatgaaagacatattggagaaaaaagttgaaaaggtggttgtgtcaaaccgattggtgacatctccatgctgtattgtcacaagcacatatggctggacagcaaacatggagagaatcatgaaagctcaagccctaagagacaactcaacaatgggttacatggcagcaaagaaacacctggagataaaccctgaccattccattattgagaccttaaggcaaaaggcagaggctgataagaacgacaagtctgtgaaggatctggtcatcttgctttatgaaactgcgctcctgtcttctggcttcagtctggaagatccccagacacatgctaacaggatctacaggatgatcaaacttggtctgggtattgatgaagatgaccctactgctgatgataccagtgctgctgtaactgaagaaatgccaccccttgaaggagatgacgacacatcacgcatggaagaagtagactaatctctggctgagggatgacttacctgttcagtactctacaattcctctgataatatattttcaaggatgtttttctttatttttgttaatattaaaaagtctgtatggcatgacaactactttaaggggaagataagatttctgtctactaagtgatgctgtgataccttaggcactaaagcagagctagtaatgctttttgagtttcatgttggtttattttcacagattggggtaacgtgcactgtaagacgtatgtaacatgatgttaactttgtggtctaaagtgtttagctgtcaagccggatgcctaagtagaccaaatcttgttattgaagtgttctgagctgtatcttgatgtttagaaaagtattcgttacatcttgtaggatctactttttgaacttttcattccctgtagttgacaattctgcatgtactagtcctctagaaataggttaaactgaagcaacttgatggaaggatctctccacagggcttgttttccaaagaaaagtattgtttggaggagcaaagttaaaagcctacctaagcatatcgtaaagctgttcaaaaataactcagacccagtcttgtggatggaaatgtagtgctcgagtcacattctgcttaaagttgtaacaaatacagatgagttaaaagatattgtgtgacagtgtcttatttagggggaaaggggagtatctggatgacagttagtgccaaaatgtaaaacatgaggcgctagcaggagatggttaaacactagctgctccaagggttgacatggtcttcccagcatgtactcagcaggtgtggggtggagcacacgtaggcacagaaaacaggaatgcagacaacatgcatcccctgcgtccatgagttacatgtgttctcttagtgtccacgttgttttgatgttattcatggaataccttctgtgttaaatacagtcacttaattccttggccttaaaa

SEQ ID NO: 46 - protein, 854 aa, Homo sapiens; identical to SEQ ID NO: 2

SEQ ID NO: 47 - DNA, 3366 bp, Homo sapiens
  CDS (191)..(2389): NM_005348 WT, CDS 191-2389
gcatgcgtaggcgcgcggccgcggcggcggctggggagggttcttccggaaggttcgggaggcttctggaaaaagcgccgcgcgctgggcgggcccgtcgctatataaggcaggcgcgggggtggcgcgtcagttgcttcagcgtcccggtgtggctgtgccgttggtcctgtgcggtcacttagccaagatgcctgaggaaacccagacccaagaccaaccgatggaggaggaggaggttgagacgttcgcctttcaggcagaaattgcccagttgatgtcattgatcatcaatactttctactcgaacaaagagatctttctgagagagctcatttcaaattcatcagatgcattggacaaaatccggtatgaaagcttgacagatcccagtaaattagactctgggaaagagctgcatattaaccttataccgaacaaacaagatcgaactctcactattgtggatactggaattggaatgaccaaggctgacttgatcaataaccttggtactatcgccaagtctgggaccaaagcgttcatggaagctttgcaggctggtgcagatatctctatgattggccagttcggtgttggtttttattctgcttatttggttgctgagaaagtaactgtgatcaccaaacataacgatgatgagcagtacgcttgggagtcctcagcagggggatcattcacagtgaggacagacacaggtgaacctatgggtcgtggaacaaaagttatcctacacctgaaagaagaccaaactgagtacttggaggaacgaagaataaaggagattgtgaagaaacattctcagtttattggatatcccattactctttttgtggagaaggaacgtgataaagaagtaagcgatgatgaggctgaagaaaaggaagacaaagaagaagaaaaagaaaaagaagagaaagagtcggaagacaaacctgaaattgaagatgttggttctgatgaggaagaagaaaagaaggatggtgacaagaagaagaagaagaagattaaggaaaagtacatcgatcaagaagagctcaacaaaacaaagcccatctggaccagaaatcccgacgatattactaatgaggagtacggagaattctataagagcttgaccaatgactgggaagatcacttggcagtgaagcatttttcagttgaaggacagttggaattcagagcccttctatttgtcccacgacgtgctccttttgatctgtttgaaaacagaaagaaaaagaacaacatcaaattgtatgtacgcagagttttcatcatggataactgtgaggagctaatccctgaatatctgaacttcattagaggggtggtagactcggaggatctccctctaaacatatcccgtgagatgttgcaacaaagcaaaattttgaaagttatcaggaagaatttggtcaaaaaatgcttagaactctttactgaactggcggaagataaagagaactacaagaaattctatgagcagttctctaaaaacataaagcttggaatacacgaagactctcaaaatcggaagaagctttcagagctgttaaggtactacacatctgcctctggtgatgagatggtttctctcaaggactactgcaccagaatgaaggagaaccagaaacatatctattatatcacaggtgagaccaaggaccaggtagctaactcagcctttgtggaacgtcttcggaaacatggcttagaagtgatctatatgattgagcccattgatgagtactgtgtccaacagctgaaggaatttgaggggaagactttagtgtcagtcaccaaagaaggcctggaacttccagaggatgaagaagagaaaaagaagcaggaagagaaaaaaacaaagtttgagaacctctgcaaaatcatgaaagacatattggagaaaaaagttgaaaaggtggttgtgtcaaaccgattggtgacatctccatgctgtattgtcacaagcacatatggctggacagcaaacatggagagaatcatgaaagctcaagccctaagagacaactcaacaatgggttacatggcagcaaagaaacacctggagataaaccctgaccattccattattgagaccttaaggcaaaaggcagaggctgataagaacgacaagtctgtgaaggatctggtcatcttgctttatgaaactgcgctcctgtcttctggcttcagtctggaagatccccagacacatgctaacaggatctacaggatgatcaaacttggtctgggtattgatgaagatgaccctactgctgatgataccagtgctgctgtaactgaagaaatgccaccccttgaaggagatgacgacacatcacgcatggaagaagtagactaatctctggctgagggatgacttacctgttcagtactctacaattcctctgataatatattttcaaggatgtttttctttatttttgttaatattaaaaagtctgtatggcatgacaactactttaaggggaagataagatttctgtctactaagtgatgctgtgataccttaggcactaaagcagagctagtaatgctttttgagtttcatgttggtttattttcacagattggggtaacgtgcactgtaagacgtatgtaacatgatgttaactttgtggtctaaagtgtttagctgtcaagccggatgcctaagtagaccaaatcttgttattgaagtgttctgagctgtatcttgatgtttagaaaagtattcgttacatcttgtaggatctactttttgaacttttcattccctgtagttgacaattctgcatgtactagtcctctagaaataggttaaactgaagcaacttgatggaaggatctctccacagggcttgttttccaaagaaaagtattgtttggaggagcaaagttaaaagcctacctaagcatatcgtaaagctgttcaaaaataactcagacccagtcttgtggatggaaatgtagtgctcgagtcacattctgcttaaagttgtaacaaatacagatgagttaaaagatattgtgtgacagtgtcttatttagggggaaaggggagtatctggatgacagttagtgccaaaatgtaaaacatgaggcgctagcaggagatggttaaacactagctgctccaagggttgacatggtcttcccagcatgtactcagcaggtgtggggtggagcacacgtaggcacagaaaacaggaatgcagacaacatgcatcccctgcgtccatgagttacatgtgttctcttagtgtccacgttgttttgatgttattcatggaataccttctgtgttaaatacagtcacttaattccttggccttaaaa

SEQ ID NO: 48 - protein, 732 aa, Homo sapiens; identical to SEQ ID NO: 4

SEQ ID NO: 49 - DNA, 2792 bp, Cricetulus griseus
  CDS (28)..(2229): NM_001246821 WT, CDS 28-2229
cgtcccgtgcgcggtcactcagcgaagatgcctgaggaaacgcagacccaagaccagccaatggaggaggaagaggtggagacctttgcctttcaggcagagatcgcccagctgatgtccttgatcatcaacaccttctactccaacaaagagatctttctgagggagctcatttcaaactcgtcagatgctctggataagatcagatacgagagtctgacagaccctagtaaattagactctgggaaggagctgcacattaatattattcccaacaaacaagaccgaacccttactatcgtggatactggaattggaatgaccaaggccgacttgatcaataaccttggtaccattgccaagtctggcaccaaagccttcatggaggctttgcaggctggtgcagacatctctatgattggccagtttggtgttggtttttacactgcgtatttggttgccgagaaagtgactgtgatcaccaaacataacgatgatgagcagtacgcctgggagtcctcagccgggggctccttcacagtgaggactgacacaggtgaaccaatgggtcgtggaacaaaggttatcttacacctgaaagaagaccaaacggagtatatggaggaaaggagaataaaggagattgtgaagaaacattctcaatttatcggctatcccattactctcttcgtggagaaggaacgcgataaggaagtcagtgatgatgaagctgaagaaaaagaagataaagaggaagagaaggaaaaggaagaaaaaggaatcgacgacaaaccagaaatagaagatgtgggttctgatgaagaggaggaggaaaagaaggatggcgacaagaagaaaaagaagaagataaaggagaagtacattgaccaagaagagctcaacaagacaaagcctatttggaccaggaatcctgatgacattactaatgaagagtatggagagttctacaagagcttaaccaacgattgggaagaacatttggcagtgaagcatttttctgttgaaggacaattggaattccgggcccttctctttgtcccaagacgtgctccatttgatctgtttgaaaacagaaagaaaaagaacaacattaagttgtatgtgcgcagagttttcatcatggataactgtgaggagttattccctgagtatctaaatttcattagaggagtggtggattctgaggatcttcctctaaatatttcccgtgaaatattgcagcaaagcaaaattttgaaagttatcagaaagaatttggtcaggaaatgcttagaactatttcatgaactggcagaagacaaagagaactacaaaaagttttatgagcagttctctaaaaatataaagcttggaattcatgaagactctcaaaatcggaagaagctttcagagctgttgcgatactatacatctgcttctggagatgagatggtttctctcaaggactattgtaccagaatgaaggaaaaccagaagcatatctacttcatcacaggtgagaccaaggaccaagttgctaactcagccttcgtggaacgtcttcggaagcatggcttagaagtaatctatatgattgagcccattgatgagtactgtgtgcaacagctgaaggagtttgagggcaagaccttggtgtctgttaccaaagaaggactggaacttccagaagatgaagaggagaaaaagaaacaggaagagaaaaagaccaaatttgaaaacctctgcaagattatgaaagatattttggagaaaaaagttgagaaggtggtcgtatcaaaccgattggtgacgtccccttgctgtattgtcacaagcacatacgggtggacagcaaacatggagagaatcattaaagctcaagctctcagagacaactcaacgatgggttacatggcagcaaagaaacacctggagataaaccctgatcactccattattgaaaccctacgacaaaaggcagaggctgacaagaatgacaagtctgtgaaggatctggtgatcttgctgtatgaaactgcactcctgtcttctggtttcagtctggaagatccccagacacatgctaacaggatctacaggatgatcaagcttggtctaggtattgatgaagatgatcctactgtggatgataccagtgctgctgtaactgaagaaatgccacccctggaaggagatgacgacacatcacgcatggaagaagtcgactaagcttcaccagagctatatgtttgatgcttactttcattccttctgataatatattttcaaggatttttgtttgatttttgttaacatttaaaacatctgtgtggcatgttttctaaggggaagaaaaatttctttctacttgtgatactgtgatactctaggcttgactcaacgggttggtagtacatttgtgtaagacaaaatgtaacctattaacttgtggtctgcagtgtttagctgttgagctgattccttagtagaccaaatttgtcacttttggaagtgttctaagatagcttcatgtttaaaaggaaaaagattaagatgggcctaagtttcatcttaaaattttcatcccctgtagttaattctgcatgtactagtcttagaagtaaatacacaagctaaaacaactgaggaattccccatgtggcttgttttcaaagtactgagaacaaaactaagcttccctaggtcttgtaagtgagcaaggcttgtgaatggaaatatagtgcccaatcacattctgctttaaaaggtaaatacagatgagataaaaacct

SEQ ID NO: 50 - protein, 733 aa, Cricetulus griseus; identical to SEQ ID NO: 6

SEQ ID NO: 51 - DNA, 2525 bp, Homo sapiens
  CDS (96)..(2240): NM_001271972 WT, CDS 96-2240
ctctcgagtcactccggcgcagtgttgggactgtctgggtatcggaaagcaagcctacgttgctcactattacgtataatccttttcttttcaagatgcctgaggaagtgcaccatggagaggaggaggtggagacttttgcctttcaggcagaaattgcccaactcatgtccctcatcatcaataccttctattccaacaaggagattttccttcgggagttgatctctaatgcttctgatgccttggacaagattcgctatgagagcctgacagacccttcgaagttggacagtggtaaagagctgaaaattgacatcatccccaaccctcaggaacgtaccctgactttggtagacacaggcattggcatgaccaaagctgatctcataaataatttgggaaccattgccaagtctggtactaaagcattcatggaggctcttcagtttggtgttggcttttattctgcctacttggtggcagagaaagtggttgtgatcacaaagcacaacgatgatgaacagtatgcttgggagtcttctgctggaggttccttcactgtgcgtgctgaccatggtgagcccattggcaggggtaccaaagtgatcctccatcttaaagaagatcagacagagtacctagaagagaggcgggtcaaagaagtagtgaagaagcattctcagttcataggctatcccatcaccctttatttggagaaggaacgagagaaggaaattagtgatgatgaggcagaggaagagaaaggtgagaaagaagaggaagataaagatgatgaagaaaaacccaagatcgaagatgtgggttcagatgaggaggatgacagcggtaaggataagaagaagaaaactaagaagatcaaagagaaatacattgatcaggaagaactaaacaagaccaagcctatttggaccagaaaccctgatgacatcacccaagaggagtatggagaattctacaagagcctcactaatgactgggaagaccacttggcagtcaagcacttttctgtagaaggtcagttggaattcagggcattgctatttattcctcgtcgggctccctttgacctttttgagaacaagaagaaaaagaacaacatcaaactctatgtccgccgtgtgttcatcatggacagctgtgatgagttgataccagagtatctcaattttatccgtggtgtggttgactctgaggatctgcccctgaacatctcccgagaaatgctccagcagagcaaaatcttgaaagtcattcgcaaaaacattgttaagaagtgccttgagctcttctctgagctggcagaagacaaggagaattacaagaaattctatgaggcattctctaaaaatctcaagcttggaatccacgaagactccactaaccgccgccgcctgtctgagctgctgcgctatcatacctcccagtctggagatgagatgacatctctgtcagagtatgtttctcgcatgaaggagacacagaagtccatctattacatcactggtgagagcaaagagcaggtggccaactcagcttttgtggagcgagtgcggaaacggggcttcgaggtggtatatatgaccgagcccattgacgagtactgtgtgcagcagctcaaggaatttgatgggaagagcctggtctcagttaccaaggagggtctggagctgcctgaggatgaggaggagaagaagaagatggaagagagcaaggcaaagtttgagaacctctgcaagctcatgaaagaaatcttagataagaaggttgagaaggtgacaatctccaatagacttgtgtcttcaccttgctgcattgtgaccagcacctacggctggacagccaatatggagcggatcatgaaagcccaggcacttcgggacaactccaccatgggctatatgatggccaaaaagcacctggagatcaaccctgaccaccccattgtggagacgctgcggcagaaggctgaggccgacaagaatgataaggcagttaaggacctggtggtgctgctgtttgaaaccgccctgctatcttctggcttttcccttgaggatccccagacccactccaaccgcatctatcgcatgatcaagctaggtctaggtattgatgaagatgaagtggcagcagaggaacccaatgctgcagttcctgatgagatcccccctctcgagggcgatgaggatgcgtctcgcatggaagaagtcgattaggttaggagttcatagttggaaaacttgtgcccttgtatagtgtccccatgggctcccactgcagcctcgagtgcccctgtcccacctggctccccctgctggtgtctagtgtttttttccctctcctgtccttgtgttgaaggcagtaaactaagggtgtcaagccccattccctctctactcttgacagcaggattggatgttgtgtattgtggtttattttattttcttcattttgttctgaaattaaagtatgcaaaataaagaatatgccgtttttataca

SEQ ID NO: 52 - protein, 714 aa, Homo sapiens; identical to SEQ ID NO: 12

SEQ ID NO: 53 - DNA, 2611 bp, Homo sapiens
  CDS (152)..(2326): NM_001271970 WT, CDS 152-2326
actctcagtctgcaaaagtgtacgcccgcagagccgccccaggtgcctgggtgttgtgtgattgacgcggggaaggaggggtcagccgatccctccccaaccctccatcccatccctgaggattgggctggtacccgcgtctctcggacagatgcctgaggaagtgcaccatggagaggaggaggtggagacttttgcctttcaggcagaaattgcccaactcatgtccctcatcatcaataccttctattccaacaaggagattttccttcgggagttgatctctaatgcttctgatgccttggacaagattcgctatgagagcctgacagacccttcgaagttggacagtggtaaagagctgaaaattgacatcatccccaaccctcaggaacgtaccctgactttggtagacacaggcattggcatgaccaaagctgatctcataaataatttgggaaccattgccaagtctggtactaaagcattcatggaggctcttcaggctggtgcagacatctccatgattgggcagtttggtgttggcttttattctgcctacttggtggcagagaaagtggttgtgatcacaaagcacaacgatgatgaacagtatgcttgggagtcttctgctggaggttccttcactgtgcgtgctgaccatggtgagcccattggcaggggtaccaaagtgatcctccatcttaaagaagatcagacagagtacctagaagagaggcgggtcaaagaagtagtgaagaagcattctcagttcataggctatcccatcaccctttatttggagaaggaacgagagaaggaaattagtgatgatgaggcagaggaagagaaaggtgagaaagaagaggaagataaagatgatgaagaaaaacccaagatcgaagatgtgggttcagatgaggaggatgacagcggtaaggataagaagaagaaaactaagaagatcaaagagaaatacattgatcaggaagaactaaacaagaccaagcctatttggaccagaaaccctgatgacatcacccaagaggagtatggagaattctacaagagcctcactaatgactgggaagaccacttggcagtcaagcacttttctgtagaaggtcagttggaattcagggcattgctatttattcctcgtcgggctccctttgacctttttgagaacaagaagaaaaagaacaacatcaaactctatgtccgccgtgtgttcatcatggacagctgtgatgagttgataccagagtatctcaattttatccgtggtgtggttgactctgaggatctgcccctgaacatctcccgagaaatgctccagcagagcaaaatcttgaaagtcattcgcaaaaacattgttaagaagtgccttgagctcttctctgagctggcagaagacaaggagaattacaagaaattctatgaggcattctctaaaaatctcaagcttggaatccacgaagactccactaaccgccgccgcctgtctgagctgctgcgctatcatacctcccagtctggagatgagatgacatctctgtcagagtatgtttctcgcatgaaggagacacagaagtccatctattacatcactggtgagagcaaagagcaggtggccaactcagcttttgtggagcgagtgcggaaacggggcttcgaggtggtatatatgaccgagcccattgacgagtactgtgtgcagcagctcaaggaatttgatgggaagagcctggtctcagttaccaaggagggtctggagctgcctgaggatgaggaggagaagaagaagatggaagagagcaaggcaaagtttgagaacctctgcaagctcatgaaagaaatcttagataagaaggttgagaaggtgacaatctccaatagacttgtgtcttcaccttgctgcattgtgaccagcacctacggctggacagccaatatggagcggatcatgaaagcccaggcacttcgggacaactccaccatgggctatatgatggccaaaaagcacctggagatcaaccctgaccaccccattgtggagacgctgcggcagaaggctgaggccgacaagaatgataaggcagttaaggacctggtggtgctgctgtttgaaaccgccctgctatcttctggcttttcccttgaggatccccagacccactccaaccgcatctatcgcatgatcaagctaggtctaggtattgatgaagatgaagtggcagcagaggaacccaatgctgcagttcctgatgagatcccccctctcgagggcgatgaggatgcgtctcgcatggaagaagtcgattaggttaggagttcatagttggaaaacttgtgcccttgtatagtgtccccatgggctcccactgcagcctcgagtgcccctgtcccacctggctccccctgctggtgtctagtgtttttttccctctcctgtccttgtgttgaaggcagtaaactaagggtgtcaagccccattccctctctactcttgacagcaggattggatgttgtgtattgtggtttattttattttcttcattttgttctgaaattaaagtatgcaaaataaagaatatgccgtttttataca

SEQ ID NO: 54 - protein, 724 aa, Homo sapiens; identical to SEQ ID NO: 8

SEQ ID NO: 55 - DNA, 2411 bp, Homo sapiens
  CDS (96)..(2126): NM_001271971 WT, CDS 96-2126
ctctcgagtcactccggcgcagtgttgggactgtctgggtatcggaaagcaagcctacgttgctcactattacgtataatccttttcttttcaagatgcctgaggaagtgcaccatggagaggaggaggtggagacttttgcctttcaggcagaaattgcccaactcatgtccctcatcatcaataccttctattccaacaaggagattttccttcgggagttgatctctaatgcttctgatgccttggacaagattcgctatgagagcctgacagacccttcgaagttggacagtggtaaagagctgaaaattgacatctccatgattgggcagtttggtgttggcttttattctgcctacttggtggcagagaaagtggttgtgatcacaaagcacaacgatgatgaacagtatgcttgggagtcttctgctggaggttccttcactgtgcgtgctgaccatggtgagcccattggcaggggtaccaaagtgatcctccatcttaaagaagatcagacagagtacctagaagagaggcgggtcaaagaagtagtgaagaagcattctcagttcataggctatcccatcaccctttatttggagaaggaacgagagaaggaaattagtgatgatgaggcagaggaagagaaaggtgagaaagaagaggaagataaagatgatgaagaaaaacccaagatcgaagatgtgggttcagatgaggaggatgacagcggtaaggataagaagaagaaaactaagaagatcaaagagaaatacattgatcaggaagaactaaacaagaccaagcctatttggaccagaaaccctgatgacatcacccaagaggagtatggagaattctacaagagcctcactaatgactgggaagaccacttggcagtcaagcacttttctgtagaaggtcagttggaattcagggcattgctatttattcctcgtcgggctccctttgacctttttgagaacaagaagaaaaagaacaacatcaaactctatgtccgccgtgtgttcatcatggacagctgtgatgagttgataccagagtatctcaattttatccgtggtgtggttgactctgaggatctgcccctgaacatctcccgagaaatgctccagcagagcaaaatcttgaaagtcattcgcaaaaacattgttaagaagtgccttgagctcttctctgagctggcagaagacaaggagaattacaagaaattctatgaggcattctctaaaaatctcaagcttggaatccacgaagactccactaaccgccgccgcctgtctgagctgctgcgctatcatacctcccagtctggagatgagatgacatctctgtcagagtatgtttctcgcatgaaggagacacagaagtccatctattacatcactggtgagagcaaagagcaggtggccaactcagcttttgtggagcgagtgcggaaacggggcttcgaggtggtatatatgaccgagcccattgacgagtactgtgtgcagcagctcaaggaatttgatgggaagagcctggtctcagttaccaaggagggtctggagctgcctgaggatgaggaggagaagaagaagatggaagagagcaaggcaaagtttgagaacctctgcaagctcatgaaagaaatcttagataagaaggttgagaaggtgacaatctccaatagacttgtgtcttcaccttgctgcattgtgaccagcacctacggctggacagccaatatggagcggatcatgaaagcccaggcacttcgggacaactccaccatgggctatatgatggccaaaaagcacctggagatcaaccctgaccaccccattgtggagacgctgcggcagaaggctgaggccgacaagaatgataaggcagttaaggacctggtggtgctgctgtttgaaaccgccctgctatcttctggcttttcccttgaggatccccagacccactccaaccgcatctatcgcatgatcaagctaggtctaggtattgatgaagatgaagtggcagcagaggaacccaatgctgcagttcctgatgagatcccccctctcgagggcgatgaggatgcgtctcgcatggaagaagtcgattaggttaggagttcatagttggaaaacttgtgcccttgtatagtgtccccatgggctcccactgcagcctcgagtgcccctgtcccacctggctccccctgctggtgtctagtgtttttttccctctcctgtccttgtgttgaaggcagtaaactaagggtgtcaagccccattccctctctactcttgacagcaggattggatgttgtgtattgtggtttattttattttcttcattttgttctgaaattaaagtatgcaaaataaagaatatgccgtttttataca

SEQ ID NO: 56 - protein, 676 aa, Homo sapiens; identical to SEQ ID NO: 10

SEQ ID NO: 57 - DNA, 2414 bp, Cricetulus griseus
  CDS (30)..(2204): XM_003501668.2 WT, CDS 30-2204
ttagtaattaatgtgtaatgctttcttagatgcctgaggaggtgcaccatggcgaggaagaggtggagacctttgccttccaggcagaaatcgcccagctcatgtccttgatcataaatactttctactcaaacaaggagattttccttcgagaattgatctccaatgcttctgatgccttggacaagattcgctatgagagcctgacagacccttccaaattggacagcggcaaagagctgaagattgacatcatccccaaccctcaggagcgcacgctgactttggtggacacgggcattggcatgaccaaagctgatctcataaataacttgggaaccattgctaagtctggcacaaaggctttcatggaggctctccaggctggtgcagacatatccatgattgggcagtttggtgttggattctactctgcctatctcgtggcagagaaagtggttgtgatcacaaagcacaatgatgacgagcagtatgcttgggagtcctctgctggtggatccttcacagtgcgtgcagaccatggtgagcccattggccggggtaccaaagtcatccttcatctcaaagaagaccagacagagtacttagaggagaggagggtcaaggaagtggtgaagaaacactcgcagttcataggctatcccatcaccctctatttggagaaggaacgagagaaggagatcagtgatgatgaggcagaagaagagaagggtgagaaagaggaagaagataaggatgatgaggaaaagccaaagattgaagatgtaggatcagatgaggaggatgacagtggcaaagataagaaaaagaaaacgaagaagattaaggagaaatacattgatcaggaagagttgaataagactaagcccatttggaccagaaaccctgatgacatcactcaagaagaatatggtgatttctataagagcctcaccaatgattgggaggaccacttggcagtcaagcacttctctgtagagggtcagttggaattcagagcattgctcttcattcctcggcgagctccctttgacctttttgagaacaagaagaagaagaacaatatcaaactgtacgtccgtcgtgtgttcatcatggacagctgtgatgagctgatccccgagtacctcaactttatccgtggcgtggtggactctgaggacctgcccctgaacatctctcgagaaatgctccaacagagcaagatcctgaaagttatccgtaaaaacattgtgaagaagtgccttgagctcttctctgagctggctgaagacaaagagaactataagaaattctacgaggccttctccaagaacttaaagcttggaatccatgaagattccactaaccgtcggcgtctctctgagctgctgcgctatcatacctctcagtctggagatgagatgacttccctgtcagaatatgtgtcccgcatgaaggagacacagaagtccatctattacatcactggtgagagcaaagagcaggtagccaactctgcctttgtggagcgtgtgccgaagcgaggctttgaagcggtgtacatgactgagcctattgatgagtactgcgtgcaacagctcaaggagtttgatggaaagagtctggtctcagtgactaaggaaggcctggagctgccagaagatgaggaagagaagaagaaaatggaggagagcaaggcaaaatttgagaatctctgcaagctcatgaaggagatcttggataagaaggttgagaaggtgaccatctccaataggctagtgtcttcaccctgctgcattgtgacaagcacctatggctggacagccaacatggagcggatcatgaaggcccaggcactcagagacaactctaccatgggctacatgatggccaaaaagcacctagagatcaaccctgaccaccccatcgtggagactctgaggcagaaggctgaggcagataaaaacgacaaagctgtcaaggatctggtggtgctgctgtttgagactgctctgctctcctctggtttctcacttgaggatccccaaacccactccaaccgcatctaccgcatgatcaaactaggcctgggtatcgatgaagatgaggtgacagcagaggagcccagtgctgctgttcctgatgagatccccccactcgagggtgatgaggatgcctcccgcatggaagaagtagattagagatcccctgggaagaccatgtcctctgtatagtttccctgagccccaccccccatgccttggctggccccaacctacctggctctctgttcaagctagaggatctctttatcctgtccttgtgccttaaggcaggaaagtcccctcccacagaatagcagggttgggtattgtgtattgtggttttgtttgttttattttgttctgaaa

SEQ ID NO: 58 - protein, 724 aa, Cricetulus griseus; identical to SEQ ID NO: 14

SEQ ID NO: 59 - DNA, 1618 bp, Homo sapiens
  CDS (64)..(1200): NM_007065 WT, CDS 64-1200
agtctccactgctgccgccgtcgccgccacccgagccggagcgggctgggccgccaaggcaagatggtggactacagcgtgtgggaccacattgaggtgtctgatgatgaagacgagacgcaccccaacatcgacacggccagtctcttccgctggcggcatcaggcccgggtggaacgcatggagcagttccagaaggagaaggaggaactggacaggggctgccgcgagtgcaagcgcaaggtggccgagtgccagaggaaactgaaggagctggaggtggccgagggcggcaaggcagagctggagcgcctgcaggccgaggcacagcagctgcgcaaggaggagcggagctgggagcagaagctggaggagatgcgcaagaaggagaagagcatgccctggaacgtggacacgctcagcaaagacggcttcagcaagagcatggtaaataccaagcccgagaagacggaggaggactcagaggaggtgagggagcagaaacacaagaccttcgtggaaaaatacgagaaacagatcaagcactttggcatgcttcgccgctgggatgacagccaaaagtacctgtcagacaacgtccacctggtgtgcgaggagacagccaattacctggtcatttggtgcattgacctagaggtggaggagaaatgtgcactcatggagcaggtggcccaccagacaatcgtcatgcaatttatcctggagctggccaagagcctaaaggtggacccccgggcctgcttccggcagttcttcactaagattaagacagccgatcgccagtacatggagggcttcaacgacgagctggaagccttcaaggagcgtgtgcggggccgtgccaagctgcgcatcgagaaggccatgaaggagtacgaggaggaggagcgcaagaagcggctcggccccggcggcctggaccccgtcgaggtctacgagtccctccctgaggaactccagaagtgcttcgatgtgaaggacgtgcagatgctgcaggacgccatcagcaagatggaccccaccgacgcaaagtaccacatgcagcgctgcattgactctggcctctgggtccccaactctaaggccagcgaggccaaggagggagaggaggcaggtcctggggacccattactggaagctgttcccaagacgggcgatgagaaggatgtcagtgtgtgacctgccccagctaccaccgccacctgcttccaggcccctatgtgccccttttcagaaaacagatagatgccatctcgcccgctcctgacttcctctacttgcgctgctcggcccagcctggggggcccgcccagccctccctggcctctccactgtctccactctccagcgcccattcaagtctctgctttgagtcaaggggcttcactgcctgcagccccccatcagcattatgccaaaggcccgggggtccggggaagggcagaggtcaccaggctggtctaccaggtagttggggagggtccccagccaaggggccggctctcgtcactgggctctgttttcactgttcgtctgctgtctgtgtcttctatttggcaaacagcaatgatcttccaataaaagatttcagatgctc

SEQ ID NO: 60 - protein, 378 aa, Homo sapiens; identical to SEQ ID NO: 16

SEQ ID NO: 61 - DNA, 1250 bp, Cricetulus griseus
  CDS (111)..(1250): XM_003499737 WT, CDS 111-1250
gaagcggaaggggcggggctccgcgagcggactctctatcccttgtgggtccctgttcagcgcccggccgtgtggagcgccgggagccaatccgggcctcctaggcgaagatggtggactacagcgtttgggatcacatcgaggtgtcggacgatgaggacgagacgcaccccaacatcgacacggccagcctcttccgctggcggcaccaggcccgagtggagcgcatggagcagtttcagaaggagaaggacgaactggaccggggctgccgtgaatgcaagcgaaaggtagccgaatgccaacgcaagctgagggagctggaagtggctgaaggcggtggccaggtggagcttgagcggctgcgagctgaggcacagcagctgcgcaaggaggagcgaagctgggagcagaagctggaggacatgcgcaagaaggagaagagcatgccctggaacgtggacaccctcagcaaggacggcttcagcaagagcatagtcaatatcaagcctgagaaggcagaggaagactcagaggaggcaagagagcagaaacacaagaccttcgttgaaaagtacgagaaacagatcaagcatttcggcatgctccaccgctgggatgacagccagaagtacctgtcagacaatgtccacctggtgtgcgaggagaccgccaactacctggttatctggtgcattgacctggaagtggaggagaaatgtgcactgatggagcaggtagctcaccagaccatggtgatgcagttcattctggagctggccaagagtctgaaggtcgatccccgtgcctgcttcaggcagttcttcaccaagatcaagaccgccgaccaacagtacatggagggcttcaaatacgaactggaggcctttaaggagcgtgtgcggggccgtgccaagctgcgcatagagaaggccatgaaggagtacgaggaggaggagcgcaagaagaggctgggccctggtggcctggaccccgtggaggtctatgagtccctgcctgaggaactgcagaagtgctttgatgtgaaggacgtgcaaatgctgcaagatgccatcagcaagatggatcccactgatgccaagtttcacatgcagcgttgcatcgattctgggctctgggtccccaactccaagtctggtgaggccaaggagggggaggaggcgggccccggggacccattgctggaagccgtccccaaagcgggcaacgagaaagacgtcagtgcgtga

SEQ ID NO: 62 - protein, 379 aa, Cricetulus griseus; identical to SEQ ID NO: 18

SEQ ID NO: 63 - DNA, 2301 bp, Homo sapiens
  CDS (118)..(1839): NM_199440 WT, CDS 1839
gccccgacgcgcaccgcgattcgccccaagggccctgcgcaggacgctgacgcgaagactcggaggcggaagaaaaaaggagctgtttctaggcttttctaggcgcccagccgagaaatgcttcggttacccacagtctttcgccagatgagaccggtgtccagggtactggctcctcatctcactcgggcttatgccaaagatgtaaaatttggtgcagatgcccgagccttaatgcttcaaggtgtagaccttttagccgatgctgtggccgttacaatggggccaaagggaagaacagtgattattgagcagagttggggaagtcccaaagtaacaaaagatggtgtgactgttgcaaagtcaattgacttaaaagataaatacaaaaacattggagctaaacttgttcaagatgttgccaataacacaaatgaagaagctggggatggcactaccactgctactgtactggcacgctctatagccaaggaaggcttcgagaagattagcaaaggtgctaatccagtggaaatcaggagaggtgtgatgttagctgttgatgctgtaattgctgaacttaaaaagcagtctaaacctgtgaccacccctgaagaaattgcacaggttgctacgatttctgcaaacggagacaaagaaattggcaatatcatctctgatgcaatgaaaaaagttggaagaaagggtgtcatcacagtaaaggatggaaaaacactgaatgatgaattagaaattattgaaggcatgaagtttgatcgaggctatatttctccatactttattaatacatcaaaaggtcagaaatgtgaattccaggatgcctatgttctgttgagtgaaaagaaaatttctagtatccagtccattgtacctgctcttgaaattgccaatgctcaccgtaagcctttggtcataatcgctgaagatgttgatggagaagctctaagtacactcgtcttgaataggctaaaggttggtcttcaggttgtggcagtcaaggctccagggtttggtgacaatagaaagaaccagcttaaagatatggctattgctactggtggtgcagtgtttggagaagagggattgaccctgaatcttgaagacgttcagcctcatgacttaggaaaagttggagaggtcattgtgaccaaagacgatgccatgctcttaaaaggaaaaggtgacaaggctcaaattgaaaaacgtattcaagaaatcattgagcagttagatgtcacaactagtgaatatgaaaaggaaaaactgaatgaacggcttgcaaaactttcagatggagtggctgtgctgaaggttggtgggacaagtgatgttgaagtgaatgaaaagaaagacagagttacagatgcccttaatgctacaagagctgctgttgaagaaggcattgttttgggagggggttgtgccctccttcgatgcattccagccttggactcattgactccagctaatgaagatcaaaaaattggtatagaaattattaaaagaacactcaaaattccagcaatgaccattgctaagaatgcaggtgttgaaggatctttgatagttgagaaaattatgcaaagttcctcagaagttggttatgatgctatggctggagattttgtgaatatggtggaaaaaggaatcattgacccaacaaaggttgtgagaactgctttattggatgctgctggtgtggcctctctgttaactacagcagaagttgtagtcacagaaattcctaaagaagagaaggaccctggaatgggtgcaatgggtggaatgggaggtggtatgggaggtggcatgttctaactcctagactagtgctttacctttattaatgaactgtgacaggaagcccaaggcagtgttcctcaccaataacttcagagaagtcagttggagaaaatgaagaaaaaggctggctgaaaatcactataaccatcagttactggtttcagttgacaaaatatataatggtttactgctgtcattgtccatgcctacagataatttattttgtatttttgaataaaaaacatttgtacattcctgatactgggtacaagagccatgtaccagtgtactgctttcaacttaaatcactgaggcatttttactactattctgttaaaatcaggattttagtgcttgccaccaccagatgagaagttaagcagcctttctgtggagagtgagaataattgtgtacaaagtagagaagtatccaattatgtgacaacctttgtgtaataaaaatttgtttaaagttaa

SEQ ID NO: 64 - protein, 573 aa, Homo sapiens; identical to SEQ ID NO: 20

SEQ ID NO: 65 - DNA, 2319 bp, Homo sapiens
  CDS (122)..(1315): NM_001539 WT, CDS 122-1315
gcggaactttccagaacgctcggtgagaggcggaggagcggtaactaccccggctgcgcacagctcggcgctccttcccgctccctcacacaccggcctcagcccgcaccggcagtagaagatggtgaaagaaacaacttactacgatgttttgggggtcaaacccaatgctactcaggaagaattgaaaaaggcttataggaaactggctttgaagtaccatcctgataagaacccaaatgaaggagagaagtttaaacagatttctcaagcttacgaagttctctctgatgcaaagaaaagggaattatatgacaaaggaggagaacaggcaattaaagagggtggagcaggtggcggttttggctcccccatggacatctttgatatgttttttggaggaggaggaaggatgcagagagaaaggagaggtaaaaatgttgtacatcagctctcagtaaccctagaagacttatataatggtgcaacaagaaaactggctctgcaaaagaatgtgatttgtgacaaatgtgaaggtagaggaggtaagaaaggagcagtagagtgctgtcccaattgccgaggtactggaatgcaaataagaattcatcagataggacctggaatggttcagcaaattcagtctgtgtgcatggagtgccagggccatggggagcggatcagtcctaaagatagatgtaaaagctgcaacggaaggaagatagttcgagagaagaaaattttagaagttcatattgacaaaggcatgaaagatggccagaagataacattccatggtgaaggagaccaagaaccaggactggagccaggcgatattatcattgtgttagatcagaaggaccatgctgtttttactcgacgaggagaagaccttttcatgtgtatggacatacagctcgttgaagcactgtgtggcttccagaagccaatatctactcttgacaaccgaaccatcgtcatcacctctcatccaggtcagattgtcaagcatggagatatcaagtgtgtactaaatgaaggcatgccaatttatcgtagaccatatgaaaagggtcgcctaatcatcgaatttaaggtaaactttcctgagaatggctttctctctcctgataaactgtctttgctggaaaaactcctacccgagaggaaggaagtggaagagactgatgagatggaccaagtagaactggtggactttgatccaaatcaggaaagacggcgccactacaatggagaagcatatgaggatgatgaacatcatcccagaggtggtgttcagtgtcagacctcttaatgggccagtgaataacactcactgctggcatttaatgtgcagtagtgaatgagtgaaggactgtaatcataatatgctcactacttgctcttgtttttgttttaataaactatagtagtgttttaaaaagttaaatgaagaataaacgcaaatataaaagctctgattttgccctgtatgtatgatgacttcagtgtgcaagatgaagtttaatacctgtaaaaactacaaagaagttcccctagcatttctaggccaaaccttgtaattgacttcagctatgtacgtggacaagcttagactgaaatgctaggtatatgtattggcttcagtgtatgacccttcattgttaagctatgaaagtaaaactctgtatttaactggcaatgaggaaaaaaaaattttgtagagaagtgttggtctgtatagttctttatattaagtgggattcattgtaatgcctctgcatttattctgttgcctcagctgttacttgaagatggcgtaatatataatttatcctgtggtatcagtgataaaaatgatacctttctgtaggaggggtttatcataatatgctgcttcttgaaggcttgcacttccagaattgtgtttccttctgctgtgccattcatatatatatacatatatatatataatcttgaccagtcctggtcatttgctcccctccttgtctgtggaccatgataagcccaagtagtgacttcagagctgggtaacagaaattaaagtgaaaagacctttacgtggagaatttgcatgcgtaatataggaaggtgttctttaggtatgttacaggattactttaaaccatttgactttcgctccaaagttatgttggtagtatagcaaattatgatgaatagctttaattgtatgtttaaaagtctcatatgttcacatgcttaaatctgggtatcagaatttaagcaattcttgaaatgtattgtctccttaatatactaattacaaagcatctccaa

SEQ ID NO: 66 - protein, 397 aa, Homo sapiens; identical to SEQ ID NO: 22

SEQ ID NO: 67 - DNA, 557 bp, Homo sapiens
  CDS (59)..(367): NM_002157 WT, CDS 59-367
gcgagtctctttgcggcgctacactagagcagagtacgagtctgaggcggagggagtaatggcaggacaagcgtttagaaagtttcttccactctttgaccgagtattggttgaaaggagtgctgctgaaactgtaaccaaaggaggcattatgcttccagaaaaatctcaaggaaaagtattgcaagcaacagtagtcgctgttggatcgggttctaaaggaaagggtggagagattcaaccagttagcgtgaaagttggagataaagttcttctcccagaatatggaggcaccaaagtagttctagatgacaaggattatttcctatttagagatggtgacattcttggaaagtacgtagactgaaataagtcactattgaaatggcatcaacatgatgctgcccattccactgaagttctgaaatctttcgtcatgtaaataatttccatatttctcttttataataaactaatgataactaatgacatccagtgtctccaaaattgtttccttgtactgatataaacacttccaaataaaaatatgtaaatga

SEQ ID NO: 68 - protein, 102 aa, Homo sapiens; identical to SEQ ID NO: 24

SEQ ID NO: 69 - DNA, 5244 bp, Homo sapiens
  CDS (323)..(2899): NM_006644 WT, CDS 323-2899
gggtcggtagttcagcgccggcgccggtgtgcgagccgcggcagagtgaggcaggcaacccgaggtgcggagcgacctgcggaggctgagccccgctttctcccagggtttcttatcagccagccgccgctgtccccgggggagtaggaggctcctgacaggccgcggctgtctgtgtgtccttctgagtgtcagaggaacggccagaccccgcgggccggagcagaacgcggccagggcagaaagcggcggcaggagaagcaggcagggggccggaggacgcagaccgagacccgaggcggaggcggaccgcgagccggccatgtcggtggtggggttggacgtgggctcgcagagctgctacatcgcggtagcccgggccgggggcatcgagaccatcgccaatgagttcagcgaccggtgcaccccgtcagtcatatcatttggatcaaaaaatagaacaatcggagttgcagccaaaaatcagcaaatcactcatgcaaacaatacggtgtctaacttcaaaagatttcatggccgagcattcaatgaccccttcattcaaaaggagaaggaaaacttgagttacgatttggttccattgaaaaatggtggagttggaataaaggtaatgtacatgggtgaagaacatctatttagtgtggagcagataacagccatgttgttgactaagctgaaggaaactgctgaaaacagcctcaagaaaccagtaacagattgtgttatttcagtcccctccttctttacagatgctgagaggcgatctgtgttagatgctgcacagattgttggcctaaactgtttaagacttatgaatgacatgacagctgttgctttgaattacggaatttataagcaggatctcccaagcctggatgagaaacctcggatagtggtttttgttgatatgggacattcagcttttcaagtgtctgcttgtgcttttaacaagggaaaattgaaggtactgggaacagcttttgatcctttcttaggaggaaaaaacttcgatgaaaagttagtggaacatttttgtgcagaatttaaaactaagtacaagttggatgcaaaatccaaaatacgagcactcctacgtctgtatcaggaatgtgaaaaactgaaaaagctaatgagctctaacagcacagaccttccactgaatatcgaatgctttatgaatgataaagatgtttccggaaagatgaacaggtcacaatttgaagaactctgtgctgaacttctgcaaaagatagaagtacccctttattcactgttggaacaaactcatctcaaagtagaagatgtgagtgcagttgagattgttggaggcgctacacgaattccagctgtgaaggaaagaattgccaaattctttggaaaagatattagcacaacactcaatgcagatgaagcagtagccagaggatgtgcattacagtgtgcaatactttccccggcatttaaagttagagaattttccgtcacagatgcagttccttttccaatatctctgatctggaaccatgattcagaagatactgaaggtgttcatgaagtctttagtcgaaaccatgctgctcctttctccaaagttctcacctttctgagaagggggccttttgagctagaagctttctattctgatccccaaggagttccatatccagaagcaaaaataggccgctttgtagttcagaatgtttctgcacagaaagatggagaaaaatctagagtaaaagtcaaagtgcgagtcaacacccatggcattttcaccatctctacggcatctatggtggagaaagtcccaactgaggagaatgaaatgtcttctgaagctgacatggagtgtctgaatcagagaccaccagaaaacccagacactgataaaaatgtccagcaagacaacagtgaagctggaacacagccccaggtacaaactgatgctcaacaaacctcacagtctcccccttcacctgaacttacctcagaagaaaacaaaatcccagatgctgacaaagcaaatgaaaaaaaagttgaccagcctccagaagctaaaaagcccaaaataaaggtggtgaatgttgagctgcctattgaagccaacttggtctggcagttagggaaagaccttcttaacatgtatattgagacagagggtaagatgataatgcaagataaattggaaaaagaaaggaatgatgctaaaaatgcagttgaggaatatgtgtatgagttcagagacaagctgtgtggaccatatgaaaaatttatatgtgagcaggatcatcaaaattttttgagactcctcacagaaactgaagactggctgtatgaagaaggagaggaccaagctaaacaagcatatgttgacaagttggaagaattaatgaaaattggcactccagttaaagttcggtttcaggaagctgaagaacggccaaaaatgtttgaagaactaggacagaggctgcagcattatgccaagatagcagctgacttcagaaataaggatgagaaatacaaccatattgatgagtctgaaatgaaaaaagtggagaagtctgttaatgaagtgatggaatggatgaataatgtcatgaatgctcaggctaaaaagagtcttgatcaggatccagttgtacgtgctcaggaaattaaaacaaaaatcaaggaattgaacaacacatgtgaacccgttgtaacacaaccgaaaccaaaaattgaatcacccaaactggaaagaactccaaatggcccaaatattgataaaaaggaagaagatttagaagacaaaaacaattttggtgctgaacctccacatcagaatggtgaatgttaccctaatgagaaaaattctgttaatatggacttggactagataaccttaaattggcctattccttcaattaataaaatatttttgccatagtatgtgactctacataacatactgaaactatttatattttcttttttaaggatatttagaaattttgtgtattatatggaaaaagaaaaaaagcttaagtctgtagtctttatgatcctaaaagggaaaattgccttggtaactttcagattcctgtggaattgtgaattcatactaagctttctgtgcagtctcaccatttgcatcactgaggatgaaactgacttttgtcttttggagaaaaaaaactgtactgcttgttcaagagggctgtgattaaaatctttaagcatttgttcctgccaaggtagttttcttgcattttgctctccattcagcatgtgtgtgggtgtggatgtttataaacaagactaagtctgacttcataagggctttctaaaaccatttctgtccaagagaaaatgactttttgctttgatattaaaaattcaatgagtaaaacaaaagctagtcaaatgtgttagcagcatgcagaacaaaaactttaaactttctctctcactatacagtatattgtcatgtgaaagtgtggaatggaagaaatgtcgatcctgttgtaactgattgtgaacacttttatgagctttaaaataaagttcatcttatggtgtcatttctaaactgttgattttgtcactaatttaaaaaatgagatgagggagaatatgaattattctagcagaaatgaagttagtgtccagtttttcttttttactgcttatgttctctcttttctaagtgaaaatgtttttctcctgacagaaaaatagcatatgtttattacattaaagcattttaaaaatactataaagtgaataaaacttaaaatcttgccacccagaagaaaacattgttaacacttcgttatacatccttggagccttttacccctaatgatgggggtatatttgtgtgagtgtctatgttatagtgctgtaggctgtttttaaaaactctgtgccagggaaattagtaaatacagtcaagtgttgtaactgcataaatgtagtgagttcattataaagacgtacttaaaaataccaatcttgctattggtagatttaggtgtttctcatttttgctgttctaaataatgctgcaatgaatctatctggttgttttgtaagcacaaaattgaagtagtgttggaggtaggggagaagacacatgcacttaggataggtgacaaccagctcctcactagggtgcaacagtttattctttttttttttttggtagagctggggtttcgctatgttgcccaagttcgtcttgaactcctgggctcaagcaatctgtctgcctcagcctcccaaagtgctgggattacatggtgtgagccaccatgcccagccatttatgatcttgatgagggccaactttccctcttccacaagggattaatcttagaactatagccaatttattataagtactatttagctactctgtgctccacacatcacggagtaatatcttcaaactatgaggtttagtaacacttgactgctgaggtttatttcctcagctctgatgcttcctgggtgaagatgtaagttattaaattaactcaaattttaaagctaacacttcattccatctagaccaggtagctcgtcatttgtacgtctgataggtgcttcaacatctcagaattggcttatttttcatgcattgcatattgtactcatttgtaatattggaatgtaaaatgttcttactaagaatctttatgtcagctattcaacatttccctactttataatttctagctgctttaccatttagcaactttaaatttttatgcagttaatatgtttctttggtttttatgttttctgaatgtctttaatgcacattaatgtatacttagtagatacacatttacacattgagaagtgaagataggtttgtgttctgtgtacaattaggacatccattaaaaaagatttttaaaaactgtgaatgggaaaacatgtttttcctcctgtcctaaaatagaacctgatgacgggagggagcatcagtcagtctggcctaaatcagtgtactgcgcttttggatgcgggcaaaagtattgtcatgttgattactttataataacgtattaatatcattggctcaaacagttgtgatatatacctagtaatcatcgaggatctcaaagatatgcaccagtttgaataaatgctgtttaaagattaaattttacaattcattttaaattgtcattttgtgacaatatttctaaacaacgtccatttttaataaca

SEQ ID NO: 70 - protein, 858 aa, Homo sapiens; identical to SEQ ID NO: 26

SEQ ID NO: 71 - DNA, 4766 bp, Homo sapiens
  CDS (1095)..(1838): NM_170735.6 WT, CDS 1095-1838
gcgcgcgcgcacacacacacacacacacagagagaacatctctagtaaaaagaaaagttgagctttcttagctagatgtgtgtattagccagaaaaagccaaggagtgaagggttttagagaactggaggagataaagtggagtctgcatatgggaggcatttgaaatggacttaaatgtctttttaatgctgactttttcagttttctccttaccagacacattgttttcatgacattagccccaggcatagacacatcattaaaatgaacatgtcaaaaaatgatttctgtttagaaataagcaaaacattttcagttgtgaccacccaggtgtagaataaagaacagtggaattgggagccctgagttctaacataaactttcttcatgacataaggcaagtcttctatggcctttggtttccttacctgtaaaacaggatggctcaatgaaattatctttcttctttgctataatagagtatctctgtgggaagaggaaaaaaaaagtcaatttaaaggctccttatagttccccaactgctgttttattgtgctattcatgcctagacatcacatagctagaaaggcccatcagacccctcaggccactgctgttcctgtcacacattcctgcaaaggaccatgttgctaacttgaaaaaaattactattaattacacttgcagttgttgcttagtaacatttatgattttgtgtttctcgtgacagcatgagcagagatcattaaaaattaaacttacaaagctgctaaagtgggaagaaggagaacttgaagccacaatttttgcacttgcttagaagccatctaatctcaggtttatatgctagatcttgggggaaacactgcatgtctctggtttatattaaaccacatacagcacactactgacactgatttgtgtctggtgcagctggagtttatcaccaagacataaaaaaaccttgaccctgcagaatggcctggaattacaatcagatgggccacatggcatcccggtgaaagaaagccctaaccagttttctgtcttgtttctgctttctccctacagttccaccaggtgagaagagtgatgaccatccttttccttactatggttatttcatactttggttgcatgaaggctgcccccatgaaagaagcaaacatccgaggacaaggtggcttggcctacccaggtgtgcggacccatgggactctggagagcgtgaatgggcccaaggcaggttcaagaggcttgacatcattggctgacactttcgaacacgtgatagaagagctgttggatgaggaccagaaagttcggcccaatgaagaaaacaataaggacgcagacttgtacacgtccagggtgatgctcagtagtcaagtgcctttggagcctcctcttctctttctgctggaggaatacaaaaattacctagatgctgcaaacatgtccatgagggtccggcgccactctgaccctgcccgccgaggggagctgagcgtgtgtgacagtattagtgagtgggtaacggcggcagacaaaaagactgcagtggacatgtcgggcgggacggtcacagtccttgaaaaggtccctgtatcaaaaggccaactgaagcaatacttctacgagaccaagtgcaatcccatgggttacacaaaagaaggctgcaggggcatagacaaaaggcattggaactcccagtgccgaactacccagtcgtacgtgcgggcccttaccatggatagcaaaaagagaattggctggcgattcataaggatagacacttcttgtgtatgtacattgaccattaaaaggggaagatagtggatttatgttgtatagattagattatattgagacaaaaattatctatttgtatatatacataacagggtaaattattcagttaagaaaaaaataattttatgaactgcatgtataaatgaagtttatacagtacagtggttctacaatctatttattggacatgtccatgaccagaagggaaacagtcatttgcgcacaacttaaaaagtctgcattacattccttgataatgttgtggtttgttgccgttgccaagaactgaaaacataaaaagttaaaaaaaataataaattgcatgctgctttaattgtgaattgataataaactgtcctctttcagaaaacagaaaaaaaacacacacacacacaacaaaaatttgaaccaaaacattccgtttacattttagacagtaagtatcttcgttcttgttagtactatatctgttttactgcttttaacttctgatagcgttggaattaaaacaatgtcaaggtgctgttgtcattgctttactggcttaggggatgggggatggggggtatatttttgtttgttttgtgtttttttttcgtttgtttgttttgttttttagttcccacagggagtagagatggggaaagaattcctacaatatatattctggctgataaaagatacatttgtatgttgtgaagatgtttgcaatatcgatcagatgactagaaagtgaataaaaattaaggcaactgaacaaaaaaatgctcacactccacatcccgtgatgcacctcccaggccccgctcattctttgggcgttggtcagagtaagctgcttttgacggaaggacctatgtttgctcagaacacattctttccccccctccccctctggtctcctctttgttttgttttaaggaagaaaaatcagttgcgcgttctgaaatattttaccactgctgtgaacaagtgaacacattgtgtcacatcatgacactcgtataagcatggagaacagtgatttttttttagaacagaaaacaacaaaaaataaccccaaaatgaagattattttttatgaggagtgaacatttgggtaaatcatggctaagcttaaaaaaaactcatggtgaggcttaacaatgtcttgtaagcaaaaggtagagccctgtatcaacccagaaacacctagatcagaacaggaatccacattgccagtgacatgagactgaacagccaaatggaggctatgtggagttggcattgcatttaccggcagtgcgggaggaatttctgagtggccatcccaaggtctaggtggaggtggggcatggtatttgagacattccaaaacgaaggcctctgaaggacccttcagaggtggctctggaatgacatgtgtcaagctgcttggacctcgtgctttaagtgcctacattatctaactgtgctcaagaggttctcgactggaggaccacactcaagccgacttatgcccaccatcccacctctggataattttgcataaaattggattagcctggagcaggttgggagccaaatgtggcatttgtgatcatgagattgatgcaatgagatagaagatgtttgctacctgaacacttattgctttgaaactagacttgaggaaaccagggtttatcttttgagaacttttggtaagggaaaagggaacaggaaaagaaaccccaaactcaggccgaatgatcaaggggacccataggaaatcttgtccagagacaagacttcgggaaggtgtctggacattcagaacaccaagacttgaaggtgccttgctcaatggaagaggccaggacagagctgacaaaattttgctccccagtgaaggccacagcaaccttctgcccatcctgtctgttcatggagagggtccctgcctcacctctgccattttgggttaggagaagtcaagttgggagcctgaaatagtggttcttggaaaaatggatccccagtgaaaactagagctctaagcccattcagcccatttcacacctgaaaatgttagtgatcaccacttggaccagcatccttaagtatcagaaagccccaagcaattgctgcatcttagtagggtgagggataagcaaaagaggatgttcaccataacccaggaatgaagataccatcagcaaagaatttcaatttgttcagtctttcatttagagctagtctttcacagtaccatctgaatacctctttgaaagaaggaagactttacgtagtgtagatttgttttgtgttgtttgaaaatattatctttgtaattatttttaatatgtaaggaatgcttggaatatctgctgtatgtcaactttatgcagcttccttttgagggacaaatttaaaacaaacaaccccccatcacaaacttaaaggattgcaagggccagatctgttaagtggtttcataggagacacatccagcaattgtgtggtcagtggctcttttacccaataagatacatcacagtcacatgcttgatggtttatgttgacctaagatttattttgttaaaatctctctctgttgtgttcgttcttgttctgttttgttttgttttttaaagtcttgctgtggtctctttgtggcagaagtgtttcatgcatggcagcaggcctgttgcttttttatggcgattcccattgaaaatgtaagtaaatgtctgtggccttgttctctctatggtaaagatattattcaccatgtaaaacaaaaaacaatatttattgtattttagtatatttatataattatgttattgaaaaaaattggcattaaaacttaaccgcatcagaagcctattgtaaatacaagttctatttaagtgtactaattaacatataatatatgttttaaatatagaatttttaatgtttttaaatatattttcaaagtacataaaa

SEQ ID NO: 72 - protein, 247 aa, Homo sapiens
MTILFLTMVISYFGCMKAAPMKEANIRGQGGLAYPGVRTHGTLESVNGPKAGSRGLTSLADTFEHVIEELLDEDQKVRPNEENNKDADLYTSRVMLSSQVPLEPPLLFLLEEYKNYLDAANMSMRVRRHSDPARRGELSVCDSISEWVTAADKKTAVDMSGGTVTVLEKVPVSKGQLKQYFYETKCNPMGYTKEGCRGIDKRHWNSQCRTTQSYVRALTMDSKKRIGWRFIRIDTSCVCTLTIKRGR

SEQ ID NO: 73 - DNA, 357 bp, Artificial Sequence
  mature BDNF WT
  CDS (1)..(357)
cacagcgacccagctagaaggggagagctgtccgtgtgcgattccatcagcgagtgggtgaccgccgctgacaagaagacagctgtggatatgagcggcggcaccgtgacagtgctggagaaggtgcccgtgtctaagggccagctgaagcagtatttctacgagaccaagtgcaaccctatgggctacacaaaggagggctgtaggggcatcgacaagcggcattggaactcccagtgtagaaccacacagtcctatgtgcgcgccctgaccatggactccaagaagaggatcggctggaggttcatccgcatcgatacaagctgcgtgtgcaccctgacaatcaagaggggccgg

SEQ ID NO: 74 - protein, 119 aa, Artificial Sequence
  Synthetic Construct
HSDPARRGELSVCDSISEWVTAADKKTAVDMSGGTVTVLEKVPVSKGQLKQYFYETKCNPMGYTKEGCRGIDKRHWNSQCRTTQSYVRALTMDSKKRIGWRFIRIDTSCVCTLTIKRGR

SEQ ID NO: 75 - protein, 25 aa, Artificial Sequence
  linker peptide
GGGGSGGGGSGGGGSGGGGSGGGGS

SEQ ID NO: 76 - protein, 5 aa, Artificial Sequence
  GS linker
GGGGS

SEQ ID NO: 77 - protein, 6 aa, Artificial Sequence
  H4 linker
EAAAAK